European Patent Specification EP 3 458 081 B1, published April 15, 2026. Title: POLYNUCLEOTIDES ENCODING CITRIN FOR THE TREATMENT OF CITRULLINEMIA TYPE 2. Applicant: MODERNATX, INC. The sequence listing filed with the application follows.

SEQUENCE LISTING (157 sequences)

SEQ ID NO: 1 - protein, 675 aa, Artificial Sequence
  wild type Citrin, isoform 1 peptide
MAAAKVALTKRADPAELRTIFLKYASIEKNGEFFMSPNDFVTRYLNIFGESQPNPKTVELLSGVVDQTKDGLISFQEFVAFESVLCAPDALFMVAFQLFDKAGKGEVTFEDVKQVFGQTTIHQHIPFNWDSEFVQLHFGKERKRHLTYAEFTQFLLEIQLEHAKQAFVQRDNARTGRVTAIDFRDIMVTIRPHVLTPFVEECLVAAAGGTTSHQVSFSYFNGFNSLLNNMELIRKIYSTLAGTRKDVEVTKEEFVLAAQKFGQVTPMEVDILFQLADLYEPRGRMTLADIERIAPLEEGTLPFNLAEAQRQKASGDSARPVLLQVAESAYRFGLGSVAGAVGATAVYPIDLVKTRMQNQRSTGSFVGELMYKNSFDCFKKVLRYEGFFGLYRGLLPQLLGVAPEKAIKLTVNDFVRDKFMHKDGSVPLAAEILAGGCAGGSQVIFTNPLEIVKIRLQVAGEITTGPRVSALSVVRDLGFFGIYKGAKACFLRDIPFSAIYFPCYAHVKASFANEDGQVSPGSLLLAGAIAGMPAASLVTPADVIKTRLQVAARAGQTTYSGVIDCFRKILREEGPKALWKGAGARVFRSSPQFGVTLLTYELLQRWFYIDFGGVKPMGSEPVPKSRINLPAPNPDHVGGYKLAVATFAGIENKFGLYLPLFKPSVSTSKAIGGGP

SEQ ID NO: 2 - DNA, 2025 bp, Artificial Sequence
  wild type Citrin, isoform 1 NA
atggcggccgccaaggtggctttaaccaagagagcagatccagctgagcttagaacaatatttttgaagtatgcaagcattgagaaaaacggtgaatttttcatgtcccccaatgactttgtcactcgatacttgaacatttttggagaaagccagcctaatccaaagactgtggaacttttaagtggagtggtggatcagaccaaagatggattaatatcttttcaagaatttgttgcctttgaatctgtcctgtgtgcccctgatgctttgtttatggtagcctttcagctgtttgacaaagctggcaaaggagaagtaacttttgaggatgttaagcaagtttttggacagaccacaattcatcaacatattccatttaactgggattcagaatttgtgcaactacattttggaaaagaaagaaaaagacacctgacatatgcggaatttactcagtttttattggaaatacaactggagcacgcaaagcaagcctttgtgcaacgggacaatgctaggactgggagagtcacagccatcgacttccgagacatcatggtcaccatccgcccccatgtcttgactccttttgtagaagaatgtctagtagctgctgctggaggtaccacatcccatcaagttagtttctcctattttaatggatttaattcgctccttaacaacatggaactcattagaaagatctatagcactctggctggcaccaggaaagatgttgaagtgactaaggaggagtttgttctggcagctcagaaatttggtcaggttacacccatggaagttgacatcttgtttcagttagcagatttatatgagccaaggggacgtatgaccttagcagacattgaacggattgctcctctggaagagggaactctgccctttaacttggctgaggcccagaggcagaaggcctcaggtgattcagctcgaccagttcttctacaagttgcagagtcggcctacaggtttggtctgggttctgttgctggagctgttggagccactgctgtgtatcctatcgatcttgtaaaaactcgaatgcagaaccaacgatcaactggctcttttgtgggagaactcatgtataaaaacagctttgactgttttaagaaagtgctacgctatgaaggcttctttggactgtatagaggtctgttgccacagttattgggagttgccccagagaaggccataaaacttacagtgaacgattttgtgagggataaatttatgcacaaagatggttcggtcccacttgcagcagaaattcttgctggaggctgcgctggaggctcccaggtgattttcacaaatcctttagaaatcgtcaagatccgtttgcaagtggcaggagaaatcaccactggtcctcgagtcagtgctctgtctgtcgtgcgggacctggggttttttgggatctacaagggtgccaaagcatgctttctgcgggacattcctttctcggccatctactttccgtgctatgctcatgtgaaggcttcctttgcaaatgaagatgggcaggttagcccaggaagcctgctcttagctggtgccatagctggtatgcctgcagcatctttagtgacccctgctgatgttatcaagacgagattacaggtggctgcccgggctggccaaaccacttacagcggagtgatagactgctttagaaagatactgcgtgaagaaggaccaaaagctctgtggaagggagctggtgctcgtgtatttcgatcctcaccccagtttggtgtaactttgctgacttacgaattgctacagcgatggttctacattgattttggaggagtaaaacccatgggatcagagccagttcctaaatccaggatcaacctgcctgccccgaatcctgatcacgttgggggctacaaactggcagttgctacatttgcagggattgaaaacaaatttggactttacctacctctcttcaagccatcagtatctacctcaaaggctattggtggaggccca

SEQ ID NO: 3 - protein, 676 aa, Artificial Sequence
  wild type Citrin, isoform 2 peptide
MAAAKVALTKRADPAELRTIFLKYASIEKNGEFFMSPNDFVTRYLNIFGESQPNPKTVELLSGVVDQTKDGLISFQEFVAFESVLCAPDALFMVAFQLFDKAGKGEVTFEDVKQVFGQTTIHQHIPFNWDSEFVQLHFGKERKRHLTYAEFTQFLLEIQLEHAKQAFVQRDNARTGRVTAIDFRDIMVTIRPHVLTPFVEECLVAAAGGTTSHQVSFSYFNGFNSLLNNMELIRKIYSTLAGTRKDVEVTKEEFVLAAQKFGQVTPMEVDILFQLADLYEPRGRMTLADIERIAPLEEGTLPFNLAEAQRQQKASGDSARPVLLQVAESAYRFGLGSVAGAVGATAVYPIDLVKTRMQNQRSTGSFVGELMYKNSFDCFKKVLRYEGFFGLYRGLLPQLLGVAPEKAIKLTVNDFVRDKFMHKDGSVPLAAEILAGGCAGGSQVIFTNPLEIVKIRLQVAGEITTGPRVSALSVVRDLGFFGIYKGAKACFLRDIPFSAIYFPCYAHVKASFANEDGQVSPGSLLLAGAIAGMPAASLVTPADVIKTRLQVAARAGQTTYSGVIDCFRKILREEGPKALWKGAGARVFRSSPQFGVTLLTYELLQRWFYIDFGGVKPMGSEPVPKSRINLPAPNPDHVGGYKLAVATFAGIENKFGLYLPLFKPSVSTSKAIGGGP

SEQ ID NO: 4 - DNA, 2028 bp, Artificial Sequence
  wild type Citrin, isoform 2 NA
atggcggccgccaaggtggctttaaccaagagagcagatccagctgagcttagaacaatatttttgaagtatgcaagcattgagaaaaacggtgaatttttcatgtcccccaatgactttgtcactcgatacttgaacatttttggagaaagccagcctaatccaaagactgtggaacttttaagtggagtggtggatcagaccaaagatggattaatatcttttcaagaatttgttgcctttgaatctgtcctgtgtgcccctgatgctttgtttatggtagcctttcagctgtttgacaaagctggcaaaggagaagtaacttttgaggatgttaagcaagtttttggacagaccacaattcatcaacatattccatttaactgggattcagaatttgtgcaactacattttggaaaagaaagaaaaagacacctgacatatgcggaatttactcagtttttattggaaatacaactggagcacgcaaagcaagcctttgtgcaacgggacaatgctaggactgggagagtcacagccatcgacttccgagacatcatggtcaccatccgcccccatgtcttgactccttttgtagaagaatgtctagtagctgctgctggaggtaccacatcccatcaagttagtttctcctattttaatggatttaattcgctccttaacaacatggaactcattagaaagatctatagcactctggctggcaccaggaaagatgttgaagtgactaaggaggagtttgttctggcagctcagaaatttggtcaggttacacccatggaagttgacatcttgtttcagttagcagatttatatgagccaaggggacgtatgaccttagcagacattgaacggattgctcctctggaagagggaactctgccctttaacttggctgaggcccagaggcagcagaaggcctcaggtgattcagctcgaccagttcttctacaagttgcagagtcggcctacaggtttggtctgggttctgttgctggagctgttggagccactgctgtgtatcctatcgatcttgtaaaaactcgaatgcagaaccaacgatcaactggctcttttgtgggagaactcatgtataaaaacagctttgactgttttaagaaagtgctacgctatgaaggcttctttggactgtatagaggtctgttgccacagttattgggagttgccccagagaaggccataaaacttacagtgaacgattttgtgagggataaatttatgcacaaagatggttcggtcccacttgcagcagaaattcttgctggaggctgcgctggaggctcccaggtgattttcacaaatcctttagaaatcgtcaagatccgtttgcaagtggcaggagaaatcaccactggtcctcgagtcagtgctctgtctgtcgtgcgggacctggggttttttgggatctacaagggtgccaaagcatgctttctgcgggacattcctttctcggccatctactttccgtgctatgctcatgtgaaggcttcctttgcaaatgaagatgggcaggttagcccaggaagcctgctcttagctggtgccatagctggtatgcctgcagcatctttagtgacccctgctgatgttatcaagacgagattacaggtggctgcccgggctggccaaaccacttacagcggagtgatagactgctttagaaagatactgcgtgaagaaggaccaaaagctctgtggaagggagctggtgctcgtgtatttcgatcctcaccccagtttggtgtaactttgctgacttacgaattgctacagcgatggttctacattgattttggaggagtaaaacccatgggatcagagccagttcctaaatccaggatcaacctgcctgccccgaatcctgatcacgttgggggctacaaactggcagttgctacatttgcagggattgaaaacaaatttggactttacctacctctcttcaagccatcagtatctacctcaaaggctattggtggaggccca

SEQ ID NO: 5 - RNA, 2025 nt, Artificial Sequence
  Citrin-CO01
auggccgccgccaagguggcgcugaccaagagggccgacccggccgagcugcggaccaucuuucugaaguacgccuccaucgagaagaacggagaguucuucaugagccccaacgauuucgugaccagguaccugaacauuuucggggagagccagcccaacccgaagaccguggagcugcucuccggcgugguggaccagaccaaggacggacugauuagcuuucaggaguucgucgcguucgaaagcgugcugugcgcccccgacgcccuguucaugguggccuuccaacuguucgacaaggccgggaaaggcgaggucacuuuugaggacgugaagcagguguucggccaaaccaccauccaccagcacauccccuucaacugggacagcgaguucgugcagcugcacuuugguaaagagaggaagcgccaucugaccuacgccgaauuuacccaguuccugcuggagauccagcuggagcacgccaagcaggccuucguccagcgcgauaacgcccggaccggccgggugaccgccaucgauuucagggacaucauggugaccauccggccccaugugcugacccccuucguggaggagugccugguggccgccgccgggggcacgacgucccaccagguguccuucuccuacuucaauggauucaacucccuccugaacaacauggagcugaucaggaagaucuacagcacccuggccggcaccaggaaagauguggaagugacgaaggaggaguucgugcuggccgcccagaaguucggccaggugacccccauggagguggacauccucuuccagcuggccgaccuguacgagcccaggggccgcaugacccuggcagauauagagcgaauugcgccccuggaggagggcacccugcccuucaaccuagccgaagcccagcgacagaaggccuccggggacuccgcccggccgguacugcugcagguggccgagagcgccuaccgguucgggcuggggagcguggccggggccgugggcgcuaccgccguguaccccauugaccuggugaagaccaggaugcagaaccagcggagcacaggcuccuucgugggcgagcugauguacaagaacagcuucgacugcuucaagaaggugcugcgcuacgagggcuucuuuggccuguacaggggccugcugccgcaacugcucggggucgcccccgagaaggccaucaagcugaccgugaaugacuucgugcgggacaaguucaugcacaaggacgggagcgugccccuggcagccgagauccuggcgggcggaugcgccggcggcagccagguaaucuucaccaacccccuggagaucgugaagauccgucugcagguggcgggcgagaucaccacgggucccagggucagcgcccugagcguggugcgggaccugggguucuucggcaucuacaagggcgccaaggccugcuuccugagggacauccccuucagcgccaucuacuuccccugcuacgcccacgugaaagccuccuuugcaaacgaggacgggcaagucagccccggcagccugcugcuggccggggccauugccggcaugcccgccgccagccuggugacccccgccgacgugaucaaaacccggcugcaggucgccgcccgagcgggccagacgaccuacuccggagucauugacugcuuccguaagauccugcgggaggaggggcccaaagcccuguggaaaggugccggcgcuaggguguuuaggagcuccccccaguuuggggucacccugcucaccuacgagcuccuccagaggugguuuuacaucgacuucgggggcgugaaacccaugggcagcgagcccgugccgaagagcaggaucaaccugcccgcgcccaaucccgaccauguggggggcuacaaacuggccguggccaccuucgccggcaucgaaaacaaguucggccucuaccugccccuguucaagcccagcgugaguaccagcaaggccaucggcggcggcccc

SEQ ID NO: 6 - RNA, 2025 nt, Artificial Sequence
  Citrin-CO02
auggccgccgccaaggucgcccugaccaagcgggccgaccccgccgagcugaggaccaucuuccucaaguacgccagcaucgaaaagaacggcgaauucuucauguccccaaacgacuucgugacccguuaccugaauaucuucggggaaagccagcccaaucccaaaaccgucgaacugcugagcggcgugguggaccagaccaaagauggacugaucagcuuucaggaguuuguggcguucgaguccgugcugugcgcccccgacgcccuguucaugguggcguuccagcuguucgauaaggcggggaaaggcgaagugaccuucgaggacgugaaacaaguguucgggcagaccaccauccaccagcacauccccuucaacugggacagcgaauuuguccaacugcacuucggcaaggagcggaagaggcaucugaccuacgccgaguucacccaguuccugcuggagauccagcuugaacaugcuaagcaggccuucgugcagagggauaacgcccggacuggcagggugaccgccaucgacuuccgggacaucauggugaccauccguccgcaugugcucacccccuucgucgaggagugccucguggccgccgccggcggaaccaccagccaccaggugagcuuuagcuacuucaacggcuuuaacagccugcucaacaacauggagcugauccguaagaucuacagcacccuggccggcacaaggaaggacgucgaggugaccaaggaggaguucgugcuggccgcccagaaguucggucaggucacccccauggagguggacauccuguuccagcucgcggaccuguacgagccccggggcaggaugacccuggccgacaucgagcggaucgccccccuggaagagggcacacuccccuucaaccuggccgaggcccagcgacagaaggccuccggcgauagcgcccggcccguccuucugcagguggccgaaagcgccuacagguucgggcugggcagcgucgccggcgccguaggcgccaccgccguguacccuaucgaccucgugaaaaccaggaugcagaaucagcggucgaccggcucuuuugucggcgagcugauguacaagaacagcuucgacugcuucaagaaagugcugagguaugagggcuucuucggccuguauaggggccugcugccccagcugcugggaguggcccccgagaaggccaucaagcugacagucaacgacuucgugagggacaaguucaugcacaaagaugggagcgugccucuggccgcggagauccuggccggcgguugcgccggcggaagccaggugaucuucaccaacccgcuggagaucgugaaaauaaggcugcaaguggccggggaaaucaccaccggcccacgcguaagcgcccugucgguggugagggaccugggcuucuucggcaucuauaagggcgccaaggccugcuuccugcgcgacauccccuucuccgccauauacuuccccugcuacgcccacgugaaggccagcuucgccaacgaggacggucaggugagccccgggagccugcugcuggcaggcgccaucgccgggaugcccgccgccagccucgugacucccgccgacgucaucaagaccaggcugcaggucgcggccagggccggccaaacgaccuacuccggcgugaucgacugcuuuaggaagauccuccgggaagaaggccccaaggcccuguggaaaggagcgggcgccaggguauuccggagcagcccacaguucggcgugacccuccucacuuacgaacugcugcagcggugguucuacaucgacuucggcggagugaaaccgauggggagcgagcccgugcccaagagcaggaucaaucugcccgcccccaaccccgaccacgugggcggguacaaacuggccguggccaccuucgccggcaucgagaacaaguucggccuguaccugccccucuucaaacccagcgucuccaccagcaaggcgaucggcgguggcccc

SEQ ID NO: 7 - RNA, 2025 nt, Artificial Sequence
  Citrin-CO03
auggccgccgccaaagucgcccugacaaagagggccgaccccgccgagcuccgcaccaucuuucugaaguacgccuccaucgagaagaacggggaguucuuuaugagccccaacgauuucgugacccgguaccugaacaucuucggcgagagccagcccaaccccaagacuguggagcugcuguccggcgugguggaccagaccaaggauggcuugauuucauuccaggaguucguggccuuugaaagcguccugugcgcccccgacgcccuguucaugguggccuuccagcuguucgauaaggccggcaagggagaggugaccuucgaggauguaaagcagguguucgggcagaccaccauccaccagcacauccccuucaacugggauagcgaauuugugcagcugcacuucggcaaagagcggaagaggcaccugaccuaugccgaguucacccaguuccugcuggagauccagcuggaacacgcaaaacaggccuuugugcagcgggacaacgccaggaccggcagggugaccgcgaucgacuucagggauaucauggugaccauuaggccgcacgugcugacacccuucguggaggagugccugguggccgccgcgggcggcaccaccucccaucagguguccuucagcuacuucaacggcuucaauagucugcugaacaacauggagcugauccggaagaucuauagcacccuggcgggcaccaggaaagacguggaagugaccaaggaggaguucgugcuggccgcccaaaaauucgggcaggugacccccauggagguggacauccucuuucagcucgccgaccuguacgagcccaggggcaggaugacccuggcggacaucgagaggaucgccccccucgaggagggcacccugcccuucaaucuggccgaggcccagaggcagaaggccuccggcgacagcgcccgccccgugcucuugcaggucgccgaguccgccuauagguucgggcugggcuccguggccggagcagugggggccaccgccguguaccccaucgaccucgugaagacgaggaugcagaaccagaggagcaccgggagcuucgugggugagcugauguacaaaaauagcuucgauugcuucaagaaggugcugagguacgagggcuucuucggccuguacagaggccugcugccacagcugcugggcguggcccccgagaaagccaucaagcucaccgucaaugacuucgucagggacaaauuuaugcacaaggacggcagcgugccccuggcugccgagauccuggcuggggggugcgccggggggagccaggugaucuucaccaacccccucgagaucgucaaaaucaggcugcagguggccggagaaauaaccacuggccccagaguguccgcccugagcguggugcgggaucugggcuucuucggcaucuauaagggcgccaaggccugcuuccugagggacauccccuucagcgccaucuauuuccccugcuacgcccacgucaaggcuagcuucgccaacgaggacggacaggugucccccggcucccugcugcucgcgggcgccaucgccgggaugcccgccgccagccuggugacccccgccgacgucaucaaaaccaggcugcaaguggccgcaagggccggccagaccaccuacuccggcgucaucgacugcuuucggaagauccugcgugaggagggccccaaggcccuguggaaaggggccggcgcccguguguuuaggagcuccccccaguucggcgugacacugcugacauaugagcugcugcaaaggugguucuacauagacuuuggcggcgugaagcccaugggcagcgagccuguccccaagagcaggaucaaccuccccgcgccgaaccccgaccacgugggcggcuacaagcucgcaguggcgaccuucgcgggaaucgagaacaaguucggacuguaccucccccuguucaagcccuccgucagcaccagcaaagcgaucggaggcggccca

SEQ ID NO: 8 - RNA, 2025 nt, Artificial Sequence
  Citrin-CO04
auggccgccgccaaaguggcccugaccaaacgugccgaccccgccgagcugcgcaccaucuuccugaaguacgccuccaucgagaagaacggcgaguucuuuaugucccccaacgacuuugucacccgguaucugaacaucuucggggagagccagcccaaccccaagaccgucgagcuccucuccggcgugguggaccagaccaaagacggccugaucagcuuccaggaguucguggccuucgaaagcgugcugugcgcgcccgacgcccuguucauggucgccuuccagcucuucgacaaagccggcaagggcgaggugaccuuugaggacgugaagcaggucuucggccaaaccaccauucaucagcacauccccuucaacugggacucugaguucgugcagcuccacuucgggaaagagaggaagcgucaccucacguacgccgaguucacccaguuucugcuggagauccagcuggagcacgccaagcaagccuuuguacagcgggacaacgcgcgcaccggccgggugacggccaucgacuucagggacaucauggucaccauccggccccacgugcugaccccguucguggaggagugucugguggccgccgccggcgggaccaccagccaccaggugaguuucuccuacuucaacggauucaacucccuccugaacaacauggagcugauccggaagaucuacagcacccuggccggcaccaggaaggacguggaggugaccaaggaagaauuugugcuggccgcccaaaaauucggccaagugacccccauggaggucgauauucuguuccagcuagccgaccucuacgagccuagggggcggaugacccuggccgacaucgagaggaucgccccccuggaagagggcacccugccuuucaaccuggccgaggcgcagcggcagaaggccucaggcgacucugcccgacccgugcuucugcaaguggccgagucggccuacagguucggacugggcagcguggccggcgccgugggcgccaccgccgucuaccccaucgaccuggucaaaaccaggaugcagaaccagaggagcacuggcuccuucguuggcgagcugauguacaagaacagcuucgacugcuucaagaagguccucagguacgagggcuucuucggccuguacagggggcuccugccccagcuucucggggucgcccccgagaaggcgaucaagcucaccgugaacgacuucgugagggauaaguucaugcacaaggacggcuccgugccccuggccgccgagauacuagccggcggcugcgccggcgguucccaggugauuuucaccaacccccuggaaaucguaaaaauccggcugcagguggccggggagauaaccaccgggccgcgcgugagcgcccugagcgugguccgggaccugggcuucuucggcaucuacaagggcgccaaggccugcuuccugagggauauccccuucuccgccaucuacuucccgugcuaugcccacgugaaagcgagcuucgccaacgaggauggccaagugagccccgggagccuccugcucgccggggccauagccggcaugcccgccgccucccucgugacgcccgccgaugugaucaagacccggcugcagguagcagcgcgggccggccagacgaccuacagcggcgugaucgacugcuuccggaaaauccugagagaggagggcccgaaggcccucuggaagggggcaggcgcacgcguguucaggagcagcccccaguucggcgugacccugcucaccuacgagcugcugcagaggugguucuauaucgacuucggcggcgugaagcccaugggcagcgaaccggugcccaaaucuaggaucaacuugcccgcacccaaccccgaccacgugggcggguacaaacuggcgguggccaccuucgccggaaucgaaaacaaguuuggccuguaccugccccuguuuaaacccuccgugagcaccagcaaggccaucgggggcggcccc

SEQ ID NO: 9 - RNA, 2025 nt, Artificial Sequence
  Citrin-CO05
auggcugccgccaagguggcccugaccaagagggccgaucccgccgagcugcgcacgaucuuccugaaguacgccagcaucgagaagaacggugaguuuuucaugagccccaacgacuucgucaccagguaucugaauaucuucggcgagucccaacccaaccccaagaccguggaacuguugagcggcgugguggaccagaccaaggacgggcucaucucguuccaggaguucguggccuucgaguccguccugugcgcccccgacgcccucuuuauggucgccuuucagcuguucgacaaggccggcaagggcgaggugacguucgaggacgugaagcaggucuucggccagaccaccauccaccagcacauccccuucaacugggacagcgaguucguacagcugcacuucggaaaggagcggaagaggcaccugaccuacgccgaguucacccaguuccugcuggagauccagcuggagcacgccaagcaggccuucgugcagcgugacaacgcgcggacgggcagggucaccgccaucgacuuccgggacauaauggugacgauccgcccccacgugcugacgcccuucguggaggagugccugguggccgccgccggcggaacaaccagccaucaggucagcuucagcuauuucaacggcuucaacucgcugcucaacaacauggaacucaucaggaagauauacagcacccuggccggcaccaggaaggacguggaggugaccaaggaagaguucguccuggccgcccagaaauuuggacaggucaccccgauggaggucgacauccuguuccagcuggccgaccucuacgagcccaggggccgcaugacccuggccgacaucgagcgcaucgccccccuggaagagggcacgcugcccuucaaccuggccgaggcccaacggcagaaggccuccggcgauagcgcccggcccguccugcuccaaguggcagaguccgccuaccguuucggccugggcuccguggccggggccgugggcgcgacugcgguguaccccaucgaccugguuaagaccaggaugcagaaucagaggagcaccggauccuuugucggggagcugauguauaagaacuccuucgacugcuucaagaaggugcugcgcuacgagggguuuuucggccuguauaggggccuccugccccagcugcugggggucgcccccgagaaggccaucaaacugaccgucaacgauuucguccgggacaaguucaugcacaaggacggcagcgugccccuggcggccgaaauccuggccggcgguugcgccggaggcucccaagugaucuucacgaacccccucgaaauugugaagauccggcugcagguggccggcgagaucaccacgggccccagggugagcgcccugagcguaguccgcgaccugggcuucuucggcaucuacaagggggcuaaagccugcuuccucagggacauccccuucuccgccaucuacuuccccuguuacgcccacgugaaggccagcuuugccaacgaggacggccaggugagccccgguagccugcuccuggccggcgccaucgcugggaugcccgccgccagccuggugacccccgccgacgucaucaagaccagguugcaggucgccgccagggccggccagaccaccuacagcggcgugauagacugcuucaggaagauccuuagggaggaggggcccaaggcgcucuggaagggggccggcgcccgcguguuccgcuccagcccccaguucggcgugacccugcugaccuaugagcuccugcagcggugguucuacaucgauuucggcggcgugaaacccaugggcagcgagcccgugcccaagagcaggaucaaccugccagcccccaaccccgaccacgugggcggguacaaacuggcgguggccacuuucgccggcauagagaacaaguucgggcuuuaccucccccuguuuaaaccuagcgugucaaccagcaaggccaucggcggcggcccc

SEQ ID NO: 10 - RNA, 2025 nt, Artificial Sequence
  Citrin-CO06
auggccgccgcaaagguugcccucacaaagcgggccgaccccgcggagcugcgaaccaucuuccugaaguacgccuccaucgagaagaacggcgaguuuuucaugagccccaacgacuuugugacccgauaccucaauaucuucggcgagagccagcccaaccccaagaccgucgagcuccucuccggcgugguggaccagaccaaagacgggcucaucagcuuccaggaguucguggccuucgaaagcgugcugugcgcccccgacgcccuguucaugguggccuuccaguuguucgauaaagccggcaagggcgaggucacguucgaagacgugaagcagguguucggacagaccaccauccaucagcacauccccuucaacugggacuccgaguucgugcagcugcacuuuggcaaggagaggaaaaggcaucugaccuacgccgaguucacccaauuucugcuggaaauccagcucgaacacgccaagcaagccuucguccaacgagauaacgccaggacaggccgcgugaccgccaucgacuucagggacaucauggugaccaucaggccccaugugcucacccccuucgucgaggagugccuaguggcggccgccgggggaaccaccagccaccaggucuccuucagcuauuucaacggcuucaacagccugcugaacaauauggagcugaucaggaagaucuacagcacccuggccggcacccggaaggacguggaggucacgaaggaggaguuuguccuggccgcccagaaguuugggcaggugaccccgauggaaguggacauccuguuccagcuggccgaucuguacgagccccggggccggaugacccuggccgauaucgagcggaucgccccccuggaggaaggcacccugcccuucaaucuggcggaggcccagagacagaaggccagcggcgacagcgccaggcccgugcucuuacagguggcagagagcgccuauagguucggccucggcuccguggccggcgccgugggggccaccgccguguacccgaucgaccuggugaagacgaggaugcagaaccagcgaaguacgggcaguuucgugggcgagcugauguacaagaacuccuucgacugcuucaagaaggugcugagguacgagggguucuucggccuguacaggggccuccugccccagcucuugggcgucgccccggagaaggccaucaagcugacggugaaugacuuugugagggacaaauucaugcauaaggacggcucugucccccuggccgccgaaauccuggccggcggcugcgcuggcggcagccaagugauuuucaccaacccccucgagaucgugaaaauuaggcugcaggucgccggggagaucaccaccgguccgcgggugagcgcccuguccgucguccgggaucugggcuucuucggcaucuacaagggagccaaggccugcuuccucagggacaucccguucagcgccaucuacuuccccugcuaugcccacgugaaagccagcuucgccaacgaggacggccaagucagcccgggcucccugcugcuggccggcgccaucgccggcaugcccgccgccagccuggugacccccgccgacgugauaaaaaccaggcugcagguggccgccagggccggccagaccaccuacagcggggucaucgacugcuuccgcaagauccuccgggaggaggggcccaaggcucuguggaagggcgccggggccagggucuucaggucgagcccccaguucggggugacgcugcugacauacgagcugcugcaaaggugguucuacaucgauuucgguggagucaaacccaugggaagcgagccgguccccaagagcaggaucaaucugcccgcccccaaccccgaccaugugggcggcuacaagcuggccguggccaccuucgccgggaucgaaaacaaguucggacuguaccugccccuguuuaaacccucaguguccaccuccaaggccaucggcggcggcccc

SEQ ID NO: 11 - RNA, 2025 nt, Artificial Sequence
  Citrin-CO07
auggccgcugccaagguggcccugaccaagcgggcugaccccgccgagcugaggacaaucuuccugaaauacgcgucgaucgagaagaacggcgaguucuucaugagcccuaacgacuucgugacccgcuaccugaacaucuucggagagagccagcccaacccgaagaccguggaacugcucagcggcgugguggaccaaaccaaggacggccugaucuccuuccaggaguucguggccuucgagagcgugcugugcgcgcccgacgcccuguuuaugguggccuuccagcuguucgauaaagcggggaagggggaggugacguucgaggaugugaagcagguguucggccagacgaccauacaccagcacauccccuucaacugggacuccgaguuugugcagcugcacuucggcaaggagcggaaaaggcauuugacguacgccgaguucacccaguuccugcuggagauccaacuggagcacgccaagcaggccuucgugcagcgagacaacgccaggaccgggagggugacggcgauagacuuccgggacaucauggugaccaucaggccccacguccugacccccuucguagaggaaugucuggucgccgccgccggcggcaccaccagccaccaagugagcuuuagcuacuucaacggcuucaacagccugcucaacaacauggaacugauccgcaagaucuacagcacccucgccggaacccgcaaggacguggaggugacgaaggaagaauucguccuggccgcacagaaguucggccaggugaccccuauggagguggauauccucuuccagcucgccgaccucuacgagccccggggcaggaugacccuggccgauaucgaaaggaucgccccccuggaggaggguacccugcccuucaaccuggccgaggcccagcggcaaaaggccuccggcgacagcgcccgacccguccugcuccaaguggccgagucagcguacagguuuggccugggcagcguggccggcgccgucggcgccaccgccguguaccccauagaccuggugaagaccaggaugcagaaccagaggagcaccggcagcuucgucggggagcugauguauaaaaacuccuuugacuguuucaagaaggugcugcgcuaugaaggcuucuucggacuguacaggggccuccugccccagcugcugggggucgcccccgagaaggccaucaagcugaccgugaacgacuuugugagggacaaguuuaugcacaaggauggcagcgugccccuggccgccgagauccuggcgggcggcugugcggggggcucgcaggucaucuucacgaauccccucgaaaucgucaaaauucgccugcaaguggccggggaaaucaccaccggaccccgcgugagcgcccucagcguggugagggaccuaggguucuucggcauuuacaagggcgccaaggccugcuuccugagggacauccccuuuuccgccaucuacuuccccuguuacgcccacgugaaggccagcuucgccaacgaggacgggcagguuagccccgggucgcugcugcuggccggcgccaucgcagggaugccggccgccagccuggucacccccgccgacgucaucaaaacccggcugcagguggccgccagggcaggccagaccaccuauagcggggugauagacugcuuucguaagauucucagggaggagggccccaaggcgcuguggaagggggccggggccagggucuuccgguccagcccccaguucggggugacacuccugaccuaugaacugcugcagaggugguucuacaucgauuucggcggcgugaagccuauggggagcgagcccgugcccaaaagcaggaucaaccugcccgccccgaaccccgaucacgugggcggauauaagcuggccguggccaccuucgccgguaucgaaaacaaguucggacuguaccugccccuguucaagcccagcgucagcaccucgaaggcgaucggaggcgguccg

SEQ ID NO: 12 - RNA, 2025 nt, Artificial Sequence
  Citrin-CO08
auggccgccgccaagguggcccugaccaagcgggccgaucccgccgagcugcguaccaucuuucugaaguacgccuccaucgagaagaacggcgaguucuucaugagccccaacgacuucgugacccgguaccucaacaucuucggugagucgcagccgaaccccaagaccguggaacuccugagcggggugguggaccagaccaaggacggccucauaagcuuccaagaguucguggccuuugaguccgugcuuugcgcccccgacgcccuguucaugguagccuuccagcuguucgacaaggccggcaaaggcgaggugaccuucgaagaugugaagcaggucuuuggucagaccaccauacaucagcacauccccuucaacugggacagcgaguuugugcagcugcauuucggaaaggagaggaaacggcaccugaccuacgccgaguucacccaguuucugcuggagauccagcuggagcacgccaaacaggccuucgugcagcgcgacaacgcgcggaccggccgggugacugccaucgacuuccgggacaucauggugacgaucaggccccacguguugacccccuucguggaggagugucugguggccgccgccggcgggaccaccucccaucaggucuccuuuagcuacuucaauggguucaacagccugcugaacaacauggagcugauccgaaagaucuauagcacgcucgccggcacccggaaggauguggaggugaccaaggaagaguucguccuggcugcccagaaguucggacaggugacccccauggagguggauauacuguuccagcucgccgaccuguacgagcccaggggacguaugacccuggcggauaucgagaggaucgccccccuggaggagggcacccugcccuucaaccuggcagaggcgcagaggcagaaggccagcggggacagcgcccgaccuguccugcugcagguggccgaauccgccuaccgguucggccugggcagcguagccggcgccgucggugccaccgccguguaccccauugaccucgugaagacccggaugcagaaccagcgaagcaccgguagcuucgucggcgagcugauguacaagaauagcuuugacugcuucaagaagguccugagguacgaaggcuuuuucggucuguaucggggccugcugccccaacugcugggggucgcccccgagaaggcuaucaagcugacggugaacgacuucgugcgcgauaaauucaugcacaaggacggcuccgucccccucgccgccgagauccuggccggaggcugcgccgggggcucccaaguuaucuucaccaacccccuggaaaucguuaagauccggcugcaggucgcgggcgagaucaccaccggcccccgcguguccgcccuguccguggugagggaccugggcuucuucggcauauacaaaggugccaaggccugcuuccugagggauauccccuucagcgccaucuacuuccccugcuacgcccacgugaaggccagcuucgccaacgaggauggccaggucucccccggcucucugcugcucgcgggcgccaucgccggcaugcccgccgcgucccuggugacccccgccgacgugauaaagaccaggcugcagguggccgccagggcaggccagaccaccuacagcggggucaucgacugcuucaggaagauccugagggaggaggggccgaaggcccucuggaagggcgccggggccaggguguuuaggucaagcccccaguucggggucacccuccugaccuacgagcugcugcagaggugguucuauaucgacuucgggggcgugaagcccaugggcuccgagccggugccaaagucccgcaucaaccugcccgccccgaaccccgaucacgucggcggcuacaagcucgccguggccaccuuugccgguaucgagaacaaguucggacuguaucugccccuguucaagccgagcgugagcaccagcaaggccaucggcgggggcccg

SEQ ID NO: 13 - RNA, 2025 nt, Artificial Sequence
  Citrin-CO09
auggccgccgccaaggucgcccugaccaagcgggcggaccccgccgagcugaggacaaucuuccugaaguacgccuccauugagaagaacggcgaauuuuucaugagccccaacgacuuugugacgcgcuaccugaauaucuucggggaaucccagcccaaccccaagacgguggagcuccugagcggcguggucgaccaaaccaaggacggacugaucagcuuucaggaguucguggccuucgagucagugcugugcgcccccgaugcccuguucaugguugccuuccagcuguucgauaaggccgguaaaggggaggugaccuucgaagaugugaagcagguguuugggcagaccaccauccaccagcauauaccguucaauugggacagcgaguuugugcagcugcacuucggcaaggagaggaagaggcaucugaccuacgccgaguucacccaauuccugcucgagauccagcucgagcacgccaagcaggccuucguacagagggacaacgcccggaccgggagggugaccgccaucgacuuccgggacaucauggugaccauccguccgcacguccugaccccuuuuguggaggagugccuggucgccgcggccggcggcaccaccagccaccaggugagcuucagcuacuucaacggguucaacagccugcucaacaacauggagcugaucaggaagaucuacagcacccuggccggcaccaggaaagacguggaggugaccaaggaggaguucgugcuggccgcccagaaguucgggcaggugacccccauggaaguggacauccuguuccaacucgccgaccuguacgagccccgagguaggaugacccuggccgacauagagcgaaucgccccgcucgaggagggaacacuccccuuuaaucuggcggaagcccaaaggcaaaaagccagcggcgacagcgcccgucccgugcugcugcagguggcggagagcgccuaucguuuugggcucgggagcguggccggcgcgguaggagccaccgccgucuaccccaucgaccuggugaagaccaggaugcagaaucagcgaagcaccggguccuucgugggcgagcugauguacaagaauagcuucgacugcuucaagaagguacugcgcuacgagggcuucuucggccuguacagggggcuccugccccagcuccugggcguugcccccgagaaggccaucaaacucaccgucaacgacuucgugagggacaaguucaugcauaaggacggcucggugccccuggccgccgaaauccuggcggggggcugcgccggaggaagccaggugaucuucacuaacccccucgagauagugaagaucaggcugcaggucgccggcgagaucaccaccggccccagggugagcgcccucuccguggugagggaucugggcuucuucggcaucuacaagggcgccaaggccugcuuccuccgggauaucccguucuccgccaucuauuuccccugcuaugcucacgugaaggccagcuuugccaacgaggauggacaggugagccccggcucccugcugcuggccggcgccaucgcagguaugcccgcugccucccucgugacccccgccgacgugaucaagacucgccuccagguggccgccagggccggccagaccaccuacuccggcgucaucgauugcuuccggaagauccuccgugaagagggucccaaggcccucuggaaaggcgccggugcgcgaguguuuaggagcagcccccaguucggggugacucugcugaccuacgagcugcuccagaggugguucuacaucgacuucggcggaguaaagcccaugggcagcgagcccguccccaagucgcgcaucaaccuccccgccccgaaccccgaccacgucggcgguuacaagcuggccguggccaccuuugccggcaucgagaacaaguucggccuguaccucccccuguucaaacccagcgugaguaccucgaaggcgaucggcggcgggccc

SEQ ID NO: 14 - RNA, 2025 nt, Artificial Sequence
  Citrin-CO10
auggcagccgccaaggucgcccuuaccaaacgugccgaucccgcggagcugaggaccaucuuccugaaguacgcaagcaucgagaagaacggcgaguucuucaugucccccaacgacuucgugaccagguaucugaauaucuucggggaaucccaacccaaucccaagaccgucgagcuccugagcggcguaguggaucaaaccaaggacggccugaucucguuccaggaguuugucgccuuugagagcgugcucugcgcccccgacgcccuguuuauggucgccuuccagcuguucgauaaggccgggaagggcgaagugaccuucgaagacgugaagcagguguucggccagaccaccauacaccagcauaucccuuuuaacugggacagcgaauucgugcagcugcacuucggaaaggagaggaagaggcaccugacguaugccgaguucacgcaauuucugcuggagauccagcucgaacacgcgaagcaggccuucguccagagggacaacgcccgcaccgggagggugaccgccaucgacuuccgcgauaucauggugaccauccgaccccacgugcugacccccuucgucgaggagugccucguggcagcagccggcggcaccacgucgcaccaggugagcuuuuccuacuucaacggguucaacagccugcugaacaauauggagcugaucaggaagauauacagcacccucgcggguacccggaaggacguggaggugaccaaggaggaguucgugcuggccgcccagaaguuugggcaggugacccccauggagguggacauccuguuccagcucgccgaccuguacgagccccggggccgcaugacccuggccgacaucgagaggaucgccccccuggaggagggcacacugccuuucaaccuggcggaggcgcagaggcagaaggccagcggggacagcgccaggcccguacugcugcaggucgccgagagcgccuaccgauuuggccuggggagcguggcuggcgcagugggcgccaccgcgguguaccccaucgaccucgugaagacccggaugcaaaaccagaggagcacagggagcuucgugggggagcugauguacaagaacagcuucgacuguuucaaaaaggugcugagguaugagggcuuuuucgggcuguacagggggcugcucccccagcugcucggcguggccccggagaaggccauaaagcugaccgugaacgacuucguccgggacaaguucaugcacaaagacggcagcgucccccuggccgccgagauccuggccggcggcugcgccggcggcucccaggugaucuuuacaaauccccucgaaauugugaagaucagguugcaaguggccggcgagaucaccaccggccccagggugagcgcccugagcguggugagggaccucggcuuuuucggcaucuacaagggcgccaaggccugcuuucugcgugacaucccauucagcgccaucuauuuccccugcuacgcccacgugaaagccucguuugccaacgaggacggccaggugucgcccggcagucugcugcuggccggugccaucgccggcaugcccgccgcgucccuggugacccccgccgacgugaucaaaacuaggcugcagguggccgcccgcgccggccagaccacguacagcggcgugaucgacugcuuccgaaagauccugagggaggagggccccaaggcccuguggaagggugcaggcgccaggguguuccgcuccuccccccaguucggcgugacgcuccugaccuacgagcugcugcagcgcugguucuauaucgauuuuggcggcgucaagcccaugggcucggagcccgugcccaaguccaggaucaaccuccccgcgcccaaccccgaccaugugggcggauacaaacucgcgguggccaccuucgcaggcaucgagaacaaguucggccucuaccugccacuuuucaagcccuccguguccaccuccaaggccaucgggggcggcccc

SEQ ID NO: 15 - RNA, 2025 nt, Artificial Sequence
  Citrin-CO11
auggccgccgccaagguggcccugaccaagagggccgaccccgcggagcugaggaccauuuuccugaaauacgccagcaucgagaagaacggcgaguucuucaugagccccaacgacuucgucacccgguaccucaacaucuucggagagagccagcccaaccccaaaacuguggagcugcugagcggcgucguggaccagacgaaggacggccucaucagcuuccaggaauucgucgccuucgaauccgugcucugcgcgcccgacgcccuguucaugguggccuuucagcuguucgacaaggcagggaagggggaagucaccuucgaggaugugaagcaaguguuuggccagacgacgauccaccagcacauccccuuuaacugggacagcgaauucgugcaacuccacuucggaaaggagcgcaagaggcaccugaccuacgcggaguucacccaauuccugcuggagauacagcuggagcacgccaagcaggcguuugugcagcgggacaacgccaggaccggcagggucaccgccaucgacuuccgggacauaauggugaccauccgcccccacgugcugacaccguucguagaagagugccugguggccgcggccgggggcacgaccucccaccaggugagcuucucguacuucaacggcuucaacagccugcucaauaacauggagcugauccggaagaucuauagcacccuggccggcaccaggaaggacguggaggugaccaaggaggaauucgugcucgcggcccagaaguucggccaggugacccccauggagguggacauccuguuucagcuggcagaccuguacgagcccaggggacguaugacccuggccgauaucgagcguaucgcgccccuggaggaggguacccuccccuucaaccuagccgaggcccagcgacagaaggccagcggggacucggcaaggcccgugcugcugcaggucgccgagagcgccuacagguuugggcuggggagcguugccggcgccgugggggccacggccguguaccccaucgaccuggucaagacccgaaugcaaaaccaacgcagcaccggcuccuucgugggggagcugauguacaaaaacuccuucgacugcuucaaaaaggugcugagguacgagggguuuuucgggcuguacaggggccugcucccccagcugcugggcguggcccccgaaaaagccaucaagcugaccgugaaugacuucgugcgcgauaaguucaugcacaaggauggguccgugccccucgcggccgagauccuggccggcgggugugccggcggcucccaggugaucuucaccaacccccuggagaucgugaaaaucaggcugcaagucgccggcgagaucaccacgggcccccgcguguccgcccugagcguggucagagaccucggcuucuucggcauauacaagggcgccaaggccugcuuccugcgggacauccccuucagcgccaucuacuuccccugcuacgcacaugugaaggcguccuucgccaaugaggacggccaggucagccccggcagccugcugcuggccggcgccaucgccggcaugcccgcagccucccucgucacccccgccgaugugaucaagaccaggcugcagguggccgcgagggcuggccagaccaccuacagcggcgugaucgacugcuucaggaagauacugagggaggaaggccccaaggcccuguggaaaggggccggcgcccgcguguucaggagcagcccccaguucggugugacccugcugacguacgagcugcugcagcggugguuuuacauagauuucggcggugugaagcccaugggcucugagcccguccccaaauccaggaucaaccugcccgcccccaaccccgaccacgugggcggcuacaagcuggccgucgccaccuucgccggcaucgagaacaaguucgggcuguaccugccccuguucaaaccgagcgugucgacaagcaaggccaucgggggcggcccc

SEQ ID NO: 16 - RNA, 2025 nt, Artificial Sequence
  Citrin-CO12
auggcggccgccaagguggcgcugacgaagcgggccgaccccgccgagcugaggaccaucuuucugaaguacgccagcaucgaaaagaacggcgaguucuucaugucccccaacgacuucgucacgagguaccugaacaucuucggagagucccaacccaauccgaagaccgucgaacugcuguccgguguggucgaccagaccaaggacggccuaaucuccuuccaggaauucguggccuucgagagcgugcugugcgcccccgaugcccuguucaugguggccuuccagcuguuugacaaagccggcaagggcgaggugacuuucgaagaugugaagcagguguuuggacagaccaccauccaccagcacauccccuucaacugggacagcgaguucgugcagcugcacuucgggaaagaacggaagaggcaucugaccuacgccgaguucacgcaguuccugcuggaaauccagcuggagcacgccaagcaagcguucgugcagagggacaacgcccggaccggcaggguuaccgccauugacuucagggauaucauggucacuauccggccccacguccugacgcccuucguggaggagugccugguggccgcggccggcgggacgaccucccaucagguguccuuuagcuacuuuaacggcuucaauagccugcugaauaauauggagcugaucaggaagaucuacuccacccuggccgggacccggaaggacguggaagugaccaaagaggaguuugugcuggccgcccagaaauucggccaggugaccccgauggagguggacaucuuguuccagcuggcggaucucuaugagccccgaggccggaugacccuggccgauauugaaaggaucgccccccuggaggagggaacccugccauucaaccucgccgaagcccagaggcagaaggcgagcggggauuccgccaggccagugcuccugcagguggcagaguccgcguaccgcuucggccuuggguccguggccggcgccgugggcgccacggcagucuaccccaucgaccuggucaagacccggaugcagaaccagcgcagcaccgggagcuucgugggcgagcugauguacaagaacagcuucgacugcuucaagaaggugcugagguacgagggguucuucgggcucuaccgggggcugcugccccagcuccuggggguggccccggagaaagccaucaagcucaccgugaaugauuuugugagggacaaguucaugcacaaggacggcagcgugccccuggccgccgagauccuggcaggcggcugcgccggcggcucccaggugaucuucaccaauccccuggagaucguuaagaucaggcuccagguggccggcgagauuaccaccggcccccgcguguccgcccugagcguggugcgcgaucugggguucuucggcaucuacaagggcgccaaggccugcuuccugcgggauauccccuucagcgccaucuacuuucccugcuaugcccaugugaaggccagcuucgcaaaugaagaugggcaggugucgcccgggucccugcugcuugccggugccaucgcgggcaugccggccgccagccuggugaccccugccgaugugaucaaaaccaggcugcagguggccgccagggccggccagaccaccuacagcggugugaucgauugcuucaggaagauccuccgggaggagggccccaaggcccuguggaagggggccggcgcccgcguguuccgcagcucgccgcaauucggugucacccuccugaccuacgagcugcugcaaaggugguucuauaucgacuucggcggcgucaagcccaugggcagcgagcccgugcccaaaucuaggaucaaccuccccgccccgaacccugaccaugucggcggcuacaagcuggccguggccaccuucgccgguaucgagaacaaguucgggcucuaccugccccuguucaagcccagcgucagcaccagcaaggccaucggcggcggcccg

SEQ ID NO: 17 - RNA, 2025 nt, Artificial Sequence
  Citrin-CO13
auggccgccgccaaaguggcccugaccaaaagggccgacccugcggagcugaggaccaucuuccugaaguacgccagcaucgagaaaaacggggaguuuuucaugagccccaacgacuucgugacgcgguaccugaacauauucggcgagagccagcccaaccccaagaccguggagcuccugagcggcguugucgaucagaccaaagauggucugaucuccuuucaggaguuuguggccuuugagagcgugcugugcgcccccgacgcccuguucauggucgccuuucagcuguucgacaaggcuggcaagggcgaggugaccuucgaggacguuaagcagguguucgggcaaaccaccauccaccagcauauccccuucaacugggacagcgaguucgugcagcuccacuucggcaaggaaaggaagcggcaccugaccuacgcagaguucacgcaguuccugcuggaaauccaacuggaacacgccaaacaggccuucguccagagggacaacgcccggacggggagggucaccgccauagacuucagggacaucauggugacgauacggccgcacgugcugacgcccuuuguggaggagugccugguggccgccgccgggggcaccaccucccaucaggugagcuucagcuauuucaauggcuucaacagccuccugaauaacauggagcuaaucaggaagauauacagcacccuggccggcaccaggaaggacguggaggugaccaaggaggaguucgugcuggccgcccaaaaguucggccaggugacccccauggaagucgauauccuguuccagcucgccgaccuguacgaaccccguggccggaugacccuggccgacaucgagcggaucgccccacuggaggagggcacucugccguucaaccuggccgaggcccaaaggcagaaagccuccggggacuccgcgaggccgguccugcugcaggucgccgagagcgccuaucgauucgggcugggcuccguggccggcgccgugggggcgaccgccguguaucccaucgaccuggugaagaccaggaugcagaaccagaggucaaccggcuccuucgugggggagcugauguauaagaauagcuucgacuguuucaagaaggugcugcgguaugaggguuucuucggccuguacagaggccugcugccccagcuguuggggguggcccccgagaaagcaaucaagcugaccgugaacgacuucgugagggacaaguucaugcacaaagacggaagcgugccccuggccgccgagauccuggccggcgguugcgcgggaggaucccaggucaucuucaccaacccgcuggagaucgucaaaauccgccugcagguggccggcgagaucaccaccggccccagggugagcgcgcuguccguggugcgggaccucggguucuucggcaucuacaaaggagccaaagccugcuuccugagggauauccccuucuccgcuaucuacuuccccuguuaugcccacgugaaggcgucguucgcuaaugaagacgggcaaguguccccagggucccugcugcucgccggcgccaucgccgguaugccagccgccagccuggugacccccgcagacgucauaaagacgcgccugcaggucgcggccagggccgggcagacaacguacagcggaguuaucgacugcuuccggaagauccuccgggaggagggccccaaggcccuguggaagggcgccggcgcucggguguuucggagcuccccgcaguucggugugacgcugcugaccuacgagcuccuccagaggugguucuacaucgacuucggcggggugaagcccaugggcuccgagcccguccccaagagccgaauaaaucugcccgcccccaaccccgaucacguggggggauacaaacuggcgguggcgaccuucgccgggaucgagaauaaguuugggcuguaccucccccuauucaagcccagcgucagcaccagcaaggccaucgggggagggccg

SEQ ID NO: 18 - RNA, 2025 nt, Artificial Sequence
  Citrin-CO14
auggccgcagccaagguggcccugaccaagcgggcugaccccgccgagcugcgcaccaucuuccugaaauacgccagcaucgaaaagaacggcgaguucuucauguccccgaacgacuucgugaccagguaucuaaacaucuucggcgaaagccaacccaaccccaagacgguggagcugcucagcggcgucguggaucagaccaaagacggccugaucuccuuccaggaguucgucgccuucgagagcgugcugugugcccccgacgcccuguucaugguggccuuccagcuguucgauaaggccggcaagggggaggugaccuucgaagacgugaagcagguuuucggucaaacgacgauccaccagcauauaccguucaauugggacuccgaguucgugcaacugcacuucgggaaggaacggaagcggcaucucaccuacgccgaguucacccaguuucugcuggaaauccagcuggaacacgccaagcaggccuucguccagagggacaacgccaggaccgggagggugaccgccaucgauuucagggacaucauggugacgaucaggccucacgugcugacgcccuucguggaggagugccuuguggccgccgccgguggcaccacuagccaccaggugagcuucagcuacuucaacggguucaacagccugcugaauaauauggagcugauaaggaagaucuauagcacccuggccggcacccggaaggauguggaggugaccaaggaggaguucgugcuggccgcccagaaguucggccaggugacacccauggaggucgacauccuguuucagcucgccgaccuguacgagcccaggggccggaugacccuggccgauaucgagaggaucgcgccccuggaggaggggacccugcccuucaaccuggcggaagcgcagcgccagaaggcaagcggagacuccgcaaggcccgugcuccugcagguggccgaaagcgcguaccgcuucggccugggguccguggccggcgcggugggcgccaccgccgucuaccccaucgaccuugucaagaccaggaugcaaaaccagcgcucgaccggcagcuucgugggcgagcucauguacaagaacagcuuugacuguuucaagaaggugcugagauaugaaggguucuucggccuguacaggggccuccugccccaacugcugggcguggcgcccgaaaaggccaucaagcucaccgugaacgacuucgugagggacaaauucaugcacaaggacggguccgucccccuggccgccgagauccuggccggcgguugcgccggcggcucccaggugaucuucaccaauccgcuggagaucgugaagauccggcugcagguggcgggcgaaaucaccaccgggccaaggguauccgcccugagcguggugcgggaccucggguucuucgggaucuacaaaggcgccaaggccugcuuccuccgcgacauccccuuuagcgcgaucuacuuccccugcuacgcccacgugaaggccuccuucgccaacgaggacggccaagugagccccggcucccugcugcuggcaggcgcgaucgccggaaugcccgccgccagccucgucacgcccgccgacgugaucaagacccggcugcaagucgccgcgagggccggccagaccaccuacagcggggucaucgauugcuuccgaaagauccugagggaggaagggcccaaggcgcuguggaagggggccggggccaggguguucagaagcagcccccaguucggcgugacccugcugaccuacgagcuccugcagcggugguucuacaucgacuucggaggcguaaagccgaugggcagcgaacccgugccuaagucccguaucaaccugcccgcccccaauccggaccacgugggcggauacaagcuggcgguggccaccuucgccggcaucgagaacaaguucggccucuaccucccgcuguuuaagcccagcgugagcaccagcaaagccaucggugguggcccg

SEQ ID NO: 19 - RNA, 2025 nt, Artificial Sequence
  Citrin-CO15
auggcugccgccaaagucgcccugaccaagcgugcggaccccgccgagcucaggacgaucuuccugaaguacgcgagcaucgagaagaacggggaguuuuucaugucccccaacgacuucgucacgagguaccugaacaucuucggcgagagccagcccaaucccaagaccguggaacugcuguccggcgugguggaccagaccaaggacgggcucaucuccuuccaggaguucguggccuucgaaagcgugcugugugcccccgaugcccuguucaugguggccuuccagcuguucgacaaggccggcaagggcgaggugaccuucgaggacgugaagcagguguucggccagaccacgauccaccagcacaucccguucaacugggacagugaguucgugcagcugcacuucggcaaagagcggaagcgccaccugaccuacgccgaguucacccaguuccuccucgagauccaacuggaacacgccaagcaggccuucgugcagcgugacaacgccaggaccggccgggugaccgccaucgauuuuagggacauaauggugaccauccgcccccacgugcugacccccuucguggaggagugccucgucgccgcggccggcggcaccaccagccaccaggugagcuucagcuacuucaacggcuucaauagccugcugaacaacauggagcugauacgaaaaaucuacagcacccuggccgggaccaggaaggacguggaagugaccaaggaggaguucguccuggccgcccagaaguucggccaagucacccccauggaaguggacauccuuuuccagcuggccgaccuguacgagccccgaggccggaugacccuggccgacaucgaacgcaucgccccccucgaggagggcacccugcccuuuaaccuggccgaggcgcagaggcagaaggccucaggagacagcgccaggccgguguugcugcagguggccgaaagcgccuacagguucggacugggcuccguggccggcgcugucggcgccaccgccguguaucccaucgaucuggugaaaacccgaaugcagaaccaaagguccaccgguagcuucgugggcgagcugauguacaaaaacagcuucgacugcuucaagaaggugcugcgguacgaaggcuucuucggccuguaccggggccugcugccccagcuccugggcgucgcccccgaaaaggcaaucaagcugaccgugaacgacuucgugcgcgacaaguucaugcacaaggacggcuccgugccccucgccgccgagauucuggccggugggugcgccggcggcagccaggugaucuucaccaacccccucgagaucgugaaaaucaggcugcaaguggccggcgagauaaccaccgggcccaggguguccgcgcugagcgucgugcgagaccugggguuuuucggcauauacaagggcgccaaggcgugcuuccugagagauauaccauucucagccaucuacuuccccugcuacgcccacguaaaggccagcuucgccaacgaggauggccaggugucccccggcagccugcugcucgccggcgcuauagccggcaugcccgccgccucccugguuacccccgccgacgucaucaaaaccaggcugcaaguugccgcccgggccggccagaccacguacagcggcgugauugauugcuuccgcaagauccugagggaagaagggcccaaagcccuguggaagggcgccggggcaaggguguuccgcagcuccccccaguucggcgugacccugcugaccuacgagcuccugcagcgcugguuuuacaucgacuucggcggcgugaagcccaugggaagcgaacccgugcccaagagcaggaucaaucugccggcccccaaccccgaccacguggggggguacaagcuggcgguggccaccuucgccgggaucgagaacaaguucggucucuaccucccccuguucaagcccucggugagcaccagcaaggcgaucgggggcggcccg

SEQ ID NO: 20 - RNA, 2025 nt, Artificial Sequence
  Citrin-CO16
auggccgccgccaagguggcccugaccaagagggccgaucccgccgagcugaggaccaucuuccugaaguacgcuagcaucgagaagaacggggaguucuucaugagcccaaacgacuuuguuacgagguaccuuaauaucuucggcgagagccaacccaaucccaagaccguggagcuccucagcgggguggucgaucagacgaaggacggccugaucagcuuucaagaguucgucgccuuugagagcguccugugcgcccccgacgcccuauucaugguggccuuccagcuguucgacaaggccggcaagggagaggugaccuucgaggacgugaaacagguguuuggucagaccacgauccaccagcacaucccguucaacugggauuccgaguucgugcagcugcacuucggcaaggagaggaagaggcaucugacguacgcugaguucacucaauuccugcuggagauccaacuggagcacgcuaagcaggccuucgugcagcgcgacaacgcccgcaccgggcgcgugaccgcuaucgacuuccgagacaucauggugaccaucaggccgcacgugcugacccccuucgucgaagagugcuugguggccgccgccggcggaaccaccagccaucaaguguccuucagcuacuucaacggcuuuaacucccugcucaauaacauggagcugaucaggaagaucuacuccacccuggccggcacgaggaaagauguagaggugaccaaggaggaguucgugcucgcggcccagaaguuugggcaggugacacccauggaaguggacauccuguuucaacuggccgaccuguacgagcccagggggaggaugacccuggccgacaucgagaggaucgccccccuggaggagggcacccugccguucaaucuggccgaggcacagaggcagaaggccuccggcgauagcgccaggcccguccugcugcagguggccgagagcgcuuauagguucgggcuggggagcguggccggagccgucggcgccaccgccguguaccccaucgaccuggucaagaccaggaugcagaaccagaggagcaccggcuccuuugugggcgagcucauguacaagaacagcuucgacugcuucaagaagguacugcgcuacgagggcuucuucggccuguacagggggcugcucccccagcugcuggggguggcgcccgagaaagccaucaaacugaccgugaacgauuucgucagggacaaguucaugcacaaggacgggagcgugccacuggccgccgagauucuggccggcgguugcgccgggggcucccaagugaucuucaccaauccccuggagaucgucaagauaaggcugcagguggccggcgaaauaaccacugggcccagggugagcgcccuguccguggugagggaccugggcuucuucggcaucuauaagggcgccaaggccugcuuccugagggacauccccuucagcgccaucuacuuccccugcuaugcucacgucaaggcaagcuucgccaacgaagacgggcaggugagccccgggagccuccuucuggccggggccaucgccggcaugcccgccgccagccuggucaccccggcggaugugaucaagaccaggcugcagguugccgcccgagccggccagaccaccuacagcggcgugaucgauuguuuucggaagauccugagggaggagggaccgaaggcacuguggaaaggggccggugccagaguguuccgauccagcccgcaguuuggagugacccugcucaccuacgagcugcuucaacggugguucuacaucgacuucggcggugugaagccaaugggcagcgagcccgugcccaagagccgcauuaaccugcccgccccaaaccccgaccacgugggcggcuacaaacuggccguggccaccuuugccggcaucgagaacaaguucggccucuaucugccccuguucaagcccagcgugucgaccagcaaggccaucggcggcgguccc

SEQ ID NO: 21 - RNA, 2025 nt, Artificial Sequence
  Citrin-CO17
auggccgccgccaagguggcccugacgaagagggccgaccccgccgaacuccggaccaucuuucugaaguacgccagcaucgagaagaacggagaguucuucaugagccccaacgauuuugugacccgguaucugaauaucuucggcgaaucccaacccaacccgaagacgguggagcugcugagcggcgugguggaccagaccaaagacgggcugaucuccuuccaggaguucguggcguuugagagcguacugugugccccggacgcccuguucaugguggccuuccagcuguucgauaaagccggcaaaggcgaggugacguucgaagacgugaaacagguguucggccagaccaccauucaccagcacauccccuucaacugggacagcgaguucguccagcugcauuuuggcaaggagcgcaagaggcaccugaccuacgccgaguucacacaauuucuccuggagauccaacuggagcacgccaagcaagccuucgugcagagggauaacgcccgaacaggccgggugaccgccaucgauuucagggacauaauggugacaauacgcccccacgugcucacccccuucguggaggagugccuaguggccgccgccggcgggacgaccucccaccaagugagcuucagcuacuuuaacggcuucaacucccugcugaauaacauggaacugauaaggaagaucuacagcacccuagccggcacccguaaggacguggaggugaccaaggaggaguucgugcuggcugcccagaaguucggccaagugacccccauggagguggacauccuguuccagcucgcggaucucuacgagccccggggccggaugacccuggcggacaucgaaaggaucgccccauuagaggagggcacccugcccuucaaucucgccgaagcccagcggcagaaggccuccggcgacagcgcgcgcccugugcuguugcagguggccgagagcgccuauagguucggccucggguccguggccggagcugugggcgccaccgccgucuacccaaucgaccuggugaagaccaggaugcaaaaucaaaggucaaccggcuccuuugugggcgagcugauguacaagaacuccuucgacugcuucaagaaggugcugagguacgaaggauucuucggccuguaccgcgggcugcugccccaacugcucggcguggcccccgagaaggccaucaagcugaccgucaacgauuucgugagggacaaguucaugcacaaggacggcagcgugccccucgccgccgagauacuggccggcgguugcgccggcggcagccaggugaucuucaccaacccccuggagaucgugaagaucaggcugcaaguggccggcgagaucaccaccggaccccgcguguccgcccugucagucgugagggaccugggguucuucggaaucuacaagggcgcaaaggccugcuuccugagggacaucccguucagcgccaucuacuuccccugcuacgcccacgucaaggccagcuucgccaaugaagacggccaggucucgcccggcagccugcugcucgccggcgccauagccggaaugccagccgccucccuggugaccccggccgacgucaucaagaccaggcuccagguggccgccagagccggccagaccaccuacagcggggugaucgacugcuucaggaagauccugcgggaggaaggccccaaggcccucuggaagggggccggggcccggguguucaggagcagcccacaguucggcgugacccugcugaccuacgagcugcuacagcggugguucuacaucgacuucgguggcgugaagcccaugggcagcgagcccgugcccaagagcaggaucaaccugcccgcccccaauccugaccaugugggcggcuacaagcuggcaguggcuaccuuugccggcaucgagaauaaguucggccuguaucugccacuguucaagcccuccgugagcaccucgaaggccauaggcggcgguccc

SEQ ID NO: 22 - RNA, 2025 nt, Artificial Sequence
  Citrin-CO18
auggccgccgccaagguggcccugaccaagagagccgaucccgccgagcugcgcaccaucuuccugaaguacgcaucaaucgagaagaacggcgaguuuuucaugagccccaacgacuuugugacgcgcuaccugaacaucuucggcgagagucagcccaaccccaaaacgguggagcugcugucaggcgugguggaccagaccaaggacggccugaucagcuuccaggaguuuguggccuuugagagcgugcugugugcccccgacgcccuguucaugguggccuuccagcuguucgacaaggcagggaagggcgaggugaccuucgaggacgugaagcagguguucgggcagaccaccauccaccagcacauccccuucaacugggacuccgaguucguccagcugcacuuuggcaaggagaggaagcgccaccugacguacgccgaguuuacccaguuccugcuggagauccaacuggagcacgccaagcaggccuucgugcagagggacaacgccaggacaggccgggugaccgccaucgacuucagggacaucauggugaccaucaggccccaugugcugaccccguucgucgaggagugccucguggccgcugccggggggaccaccagccaccaggugagcuuuaguuacuucaauggcuuuaacucgcugcugaacaacauggagcugauccggaagauauacagcacccuggccggaacccggaaggacguggaagucaccaaagaggaguucgugcuggccgcccagaaguuuggccaagugacgcccauggaggucgacauccuguuccagcuggccgaccuauacgagccccgaggccggaugacccuggccgacauagaaaggauagccccccuggaggaggggacccuucccuucaaucuggccgaggcccagaggcagaaggccagcggcgauagcgccaggcccgugcuacugcagguggccgagagugccuaccgguucggccugggcuccguggcaggcgccgugggcgccaccgccguguacccgaucgaccuggugaagaccaggaugcagaaccagcggagcaccggguccuucgugggggagcugauguacaagaacuccuucgacuguuuuaagaaagugcugcgcuacgagggguuuuucgggcuguaccgaggccugcugccccagcuucucggcguggccccggagaaggcuauaaagcugaccgugaaugauuucgugagggacaaguucaugcacaaggacggcagcguaccucucgcggccgagauccucgccggcggcugugcgggcgggagccaggugaucuuuaccaacccgcuggagauugugaagauucggcugcagguggcgggcgaaauuaccaccggccccaggguaucggcccuguccguggugagggaccugggcuucuuuggcaucuacaagggggccaaggccuguuuccucagggauauccccuucagcgccaucuacuuccccugcuacgcccacgugaaggccuccuuugccaacgaggacggccaggugagccccggcagccugcuucuggccggcgccaucgccggcaugcccgccgccagccuggugaccccggcggacgugaucaagacgcgccugcagguggcagcaagggccgggcagaccaccuacagcggggugaucgauugcuucaggaagauccugagggaggaaggccccaaggcccucuggaagggggccggagccaggguguuccggagcuccccgcaguucggcgugacccugcugaccuaugagcuccugcagcggugguucuacauagacuucggcggagugaagccuaugggcagcgagcccgugccgaaaagcaggaucaaccugcccgccccgaaccccgaccaugucggcggcuacaagcuggcgguggccaccuucgcagggauagagaauaaguuuggccuguaccugccccucuucaagcccagcgugagcaccagcaaggccauaggcggcgggccc

SEQ ID NO: 23 - RNA, 2025 nt, Artificial Sequence
  Citrin-CO19
auggccgccgccaagguggcucugaccaagagggcggaccccgccgagcugaggaccaucuuccugaaguacgccucuaucgagaagaacggcgaauucuucaugucacccaacgacuucgugaccagguaccugaacaucuucggcgagagccaacccaaccccaagaccguggagcugcugagcggcgugguggaccagacgaaggacggccugaucagcuuccaggaguucguggccuucgagagcgugcucugcgcccccgacgcccuguucaugguggccuuccagcuguucgacaaggccggcaagggcgaagugaccuucgaagacgugaagcagguguuuggccagaccaccauccaccagcacauccccuucaacugggacagcgaauucguccagcugcacuucggcaaggagcggaagcggcaccucaccuacgccgaguucacccaguuucugcucgagauccagcuggaacacgccaagcaagccuucgugcaaagggauaacgccaggaccggcagggucaccgccaucgacuuccgugacaucauggucaccauacgaccccacgugcugacccccuucgucgaggagugucugguggccgccgcaggggggacgaccagccaccaaguaagcuucagcuacuucaacggcuucaacagccugcugaacaacauggagcucaucagaaaaaucuacucuacccuggccgggaccaggaaagacgucgaagugacgaaggaggaguucguccuggccgcccagaaguucggccaggucacccccauggaggucgacauacuguuccagcuggccgaccucuaugaacccaggggcaggaugacccuggccgauaucgaacgcaucgccccccuggaggaggggaccuugccauucaaucuggccgaggcccagcggcagaaggccagcggcgacagcgccagacccgugcugcugcaggucgcggagagcgccuaccguuucggccuggggagcguagcgggcgccgugggggccaccgccguguaccccaucgaucuggugaagaccaggaugcagaaccagcgauccaccggcagcuucgugggcgagcugauguauaagaacucauuugacugcuucaagaaggugcuucgauacgagggguucuucggccuguaccgaggacugcugccccaacugcugggcguggccccggagaaggcgauuaagcugaccgugaaugauuucgugcgcgacaaauucaugcacaaggacggcuccgugccccuggccgccgaaauccuggccggcgggugcgccgguggcucccaggugauauucaccaauccccucgaaaucguaaaaaucaggcugcagguggcgggggagaucaccaccgggccgagggugagcgcccugucagugguaagggaccugggguucuucggcaucuacaagggagccaaggccugcuuccugcgggauaucccauucagcgccauuuauuuccccugcuacgcccaugugaaggccuccuucgccaacgaggacggccaagugagccccggcagccugcugcuggccggggccaucgccggcaugcccgccgccucgcuagugacccccgccgaugucaucaagacccggcugcagguggccgccagggccggucagacgaccuacucaggcgugaucgacugcuuuaggaaaauccugagggaggagggccccaaagcgcuguggaagggcgcuggggcccgugucuucagguccuccccccaguucggagugacccugcucacguacgaacugcugcagaggugguuuuacaucgacuucggcggcgugaagcccaugggcagcgagcccgugcccaaaagcaggaucaaccucccggcgcccaaccccgaccauguggggggcuacaaacuggcgguggccacguucgcgggcaucgagaacaaguucgggcuguaccugccccuguucaaacccagcgugagcaccagcaaggccaucggcggcggucca

SEQ ID NO: 24 - RNA, 2025 nt, Artificial Sequence
  Citrin-CO20
auggccgccgccaaggucgcccucaccaaaagggccgacccggccgagcuccggaccauuuuccucaaguacgccagcaucgaaaagaacggcgaguucuucaugagccccaacgacuucguaacaagguaccucaacaucuucggugagagccagcccaaccccaagaccguggagcuccucagcggcguggucgaucagaccaaggauggccugaucagcuuucaagaguucguggccuucgagagcguauugugcgcccccgacgcgcuguuuaugguggccuuucagcuguucgacaaagccggcaaaggcgaggugacauucgaggacgugaagcaaguguucggccaaaccaccauccaccaacacauccccuucaacugggacuccgaguucgugcagcugcacuucgguaaggagcggaagcgccaucugacuuacgccgaguucacgcaauuccuccuggagauccagcuggagcacgccaagcaggccuuugugcaacgagacaacgccaggaccgguagggucaccgccaucgauuuccgggacaucaugguaacgauacggccccacgugcugacgccguuuguggaagagugucuaguagccgcggccggcggcaccaccucgcaccaggucagcuucagcuacuucaauggcuucaauagccugcucaacaacauggagcugaucaggaagaucuauagcacccucgccggcaccaggaaggacguggaagugaccaaggaagaguucgugcuggccgcgcagaaguucggccaggugacccccauggaagucgacauccuguuccagcuggccgaccuguacgagccccgggggaggaugacccuggcggacaucgagaggaucgccccccuggaggaggggacccugccguucaaccuggcagaggcccagaggcaaaaggccagcggggacagcgcccggcccgugcugcugcaaguggccgagagcgccuaccgauucggccuugggagcgucgccggcgccgugggggcgaccgccguguaucccaucgaccuggugaaaacccgaaugcagaaccagcggagcaccggauccuuugugggcgagcugauguacaagaacagcuucgacugcuucaagaagguccugcgcuaugagggcuucuucggccuguacagagggcugcugccccagcuccuggggguggcccccgaaaaagccaucaagcugaccgucaacgacuuugugagggauaaguuuaugcacaaagacggcagcgugccccucgccgccgagauccuggccggaggcugcgccggagguagccaggugaucuucaccaauccccuggagauagugaaaauccggcugcagguggccggcgaaaucaccaccggccccaggguguccgcccuguccguggugcgcgaccugggcuucuucggcaucuauaagggcgccaaggcgugcuuccucagggacaucccauucagcgccauauauuuccccugcuacgcccacgugaaggccuccuucgccaacgaggacggccaggugagccccggcucgcugcugcuggccggagccaucgccggcaugcccgccgccucacuggugacccccgcggacgugauaaagacccggcugcagguggccgcgagggccggacagaccaccuacuccggggucaucgacugcuucaggaagauccuccgggaggagggccccaaggcccuguggaaaggagcgggcgccaggguguuucgaagcagcccccaguucggcgugacccuccugaccuacgagcugcuccagaggugguucuacaucgacuucgggggcgugaagcccaugggcuccgagcccgugcccaagagcaggauuaaccugccggcccccaacccagaccacgucggcggcuacaagcuggccguggccaccuuugcaggcaucgaaaacaaguuuggccucuaccuuccccuguuuaaacccagcgugagcacaagcaaggccauuggggggggaccg

SEQ ID NO: 25 - RNA, 2025 nt, Artificial Sequence
  Citrin-CO21
auggccgccgccaaaguggcccugacgaagagggcagaccccgccgagcugaggaccaucuuucugaaguacgcaagcaucgagaagaacggcgaguucuucaugagccccaacgacuucgugaccagguaccuuaauaucuucggcgagagccagcccaaccccaaaacgguggagcugcucagcgggguggucgaccagaccaaagacggacugaucagcuuccaggaguucguggccuucgaguccgugcugugcgccccagaugcccuguucaugguggccuuccaacucuucgacaaggccgggaagggcgaagugaccuucgaagacgugaagcagguguucgggcaaacaacgauccaccagcauauccccuucaacugggacucggaguucgugcagcugcauuucggcaaagagaggaagcgccaucuaacuuacgccgaguucacccaguuccugcuggaaauccagcuggagcaugccaagcaggccuucguccagcgcgauaacgcccgaaccggccgcgugaccgccauugacuucagggacaucauggugaccauccgcccccacgugcugacccccuuugucgaggagugccugguggccgccgccggggggacgaccucccaccaggucagcuucuccuauuucaacggcuucaacagccugcugaacaauauggagcugaucaggaagaucuacagcacccucgccggcacccgcaaggauguggaggugacaaaggaggaguucgugcuggccgcccaaaaguucggucaggugaccccgauggagguggacauccucuuccaacuggccgaccuguacgagccccguggccgcaugacccucgccgauaucgagaggaucgccccccuggaggagggcacccugcccuucaaucuggccgaggcccagcggcagaaggcguccggcgauagcgcgcgcccaguccuccuccaggucgccgagucggcauaccguuucggccucggaagcguggccggcgccgugggugccaccgccguguaccccaucgaccuggugaagaccaggaugcagaaccagaggagcaccggaagcuucgugggggagcugauguacaagaacagcuuugacugcuucaaaaaggugcugcgauacgagggauuuuuuggccucuacaggggccugcugccccagcugcugggagucgcccccgagaaggccaucaagcugaccgugaacgacuucgugagggacaaguucaugcauaaggacggcuccgucccccuggccgccgagauccuggcaggggggugcgccggcggcucccaggucaucuuuaccaacccccuggagaucgugaagauaaggcugcagguggccggcgaaaucaccaccgggcccagggucagcgcccugagcguggugcgggaccugggcuuuuuuggcaucuacaaaggcgccaaggccugcuuccugcgagacauccccuucucagccaucuacuuccccugcuacgcccaugugaaggccaguuucgccaaugaggacggccagguguccccaggcagccuucugcucgccggcgccaucgccggcaugcccgccgccucccuggugaccccggcggacgugaucaagaccaggcugcagguggccgccagggcuggucagacgaccuacagcggcgugaucgacugcuucaggaagauccucagggaggagggccccaaagcccuguggaagggcgcaggcgccagaguguucaggagcagcccccaguucggggugacccugcucaccuacgagcugcugcagaggugguucuacaucgacuucggcggugugaaacccaugggcagcgaacccguacccaaaagccggaucaaccugcccgcccccaaucccgaccacguggggggguacaagcucgccguggccacauucgcggggaucgagaacaaguucgggcucuaccugccccuguuuaaaccgagcgugagcacgagcaaggccaucggcggggggccc

SEQ ID NO: 26 - RNA, 2025 nt, Artificial Sequence
  Citrin-CO22
auggccgccgccaaagucgcccugacgaagagggcggaucccgccgagcucaggacaaucuuccugaaguacgcguccaucgagaagaacggggaguucuucaugucccccaacgacuucgugaccagguaccuaaacaucuucggcgagucccagcccaaccccaagaccguggagcugcuguccggagugguggaccagaccaaggacggccugaucagcuuccaagaauucgucgccuuugagagcgugcugugcgccccggacgcccuguucaugguggccuuccagcuguucgacaaagccgguaagggcgaggugaccuucgaggaugugaagcagguguucgggcagaccacaauccaccaacacaucccguucaauugggacagcgaguuugugcagcugcacuucgguaaggagcggaagcgucaucugacguacgcggaguucacccaguuccugcuggagauccagcuggagcaugccaagcaggccuucgugcagagggacaacgcccggacaggcagggugacugcgauugacuuccgagauaucauggugaccaucaggccacacguccugacccccuucguggaggagugucucgucgccgccgcggguggcacgaccagccaccaggucagcuucagcuacuucaacggcuucaacucacugcugaacaacauggaguugauucggaaaaucuacagcacccuggccggcaccaggaaggaugucgaagucaccaaggaggaguucgugcuggccgcccagaaguucggccaggugaccccaauggagguggauauccuguuccagcuggccgaccucuacgagccccggggaaggaugacccuggccgauaucgagcgcaucgccccccuggaagagggcacccugccauucaaccuggccgaggcccagcgucagaaggccagcggggauucagccaggcccguacugcugcagguggccgagagcgccuaccgguucggccugggcuccguggccggcgccgugggcgccaccgccguuuacccgaucgaccucgugaagacccggaugcagaaccaacgcucgaccggcagcuuugugggcgagcugauguacaagaacagcuuugacugcuucaagaaagugcugagguacgagggcuuuuuuggccuguaccggggccugcugccccaacuccugggcguggcccccgagaaggccaucaagcugaccgugaacgacuucguccgggacaaguucaugcacaaggacggguccgucccccuggcggccgagauccuggccgguggcugugccggcggcucccaggugaucuucaccaacccccuggagaucgucaagaucaggcugcagguggcaggcgagaucaccaccggcccgcgagucagcgccuugagcguggucagggaucugggcuucuucgguaucuacaaaggcgccaaggcgugcuuccuccgggauaucccguucuccgccaucuauuuucccugcuacgcccacgugaaggcuagcuucgccaacgaggacgggcaagucagccccggcagccuccuccuggccggagccaucgccgggaugcccgccgccagccuggugacccccgccgacgugaucaagacgaggcuccagguggccgccagggccgggcagacgacguacuccggcgugaucgacugcuuccgcaagauucugagggaggagggccccaaagcccuguggaagggggccggcgcccggguguuccggagcuccccgcaguucggggugacccuccugaccuacgaacugcugcagcggugguucuacaucgacuucggcggagugaagcccauggguagcgagccugugcccaaaagcagaaucaaccuccccgcccccaaccccgaccacgucgggggcuacaagcucgccguggcgaccuucgccggcaucgaaaacaaguucggccucuaccucccccuguucaagccauccgucagcaccagcaaagccaucgggggaggcccc

SEQ ID NO: 27 - RNA, 2025 nt, Artificial Sequence
  Citrin-CO23
auggccgccgccaaggucgcccugaccaaacgggccgaccccgccgaacugcggaccaucuuccucaaguacgccagcaucgaaaagaacggcgaauucuucaugucccccaacgacuucgucaccagguaccugaacaucuucggcgaaucccaacccaaccccaagaccguggagcugcugagcggcguggucgaccagacaaaggaugggcucaucuccuuucaggaguucgucgccuucgaaagcgugcugugcgcccccgacgcccuguucaugguggccuuccagcuguucgacaaggccgggaagggcgaggugaccuuugaggacgugaagcagguguuugggcagaccacgauccaccagcacaucccauuuaacugggacagcgaguucgugcagcugcacuucggcaaggaacgcaagcgccaccugacguacgcugaguuuacucaguuccugcuggagauccagcuggaacacgccaagcaggccuucgugcagagggauaaugcgcgcaccggaagggucaccgccaucgacuucagggacaucauggugaccaucaggccccacguccugacccccuucguagaggagugucugguggccgccgccggcgggaccacgucccaccagguuagcuuuuccuacuucaacggcuucaacucccugcugaacaacauggagcugaucaggaagaucuauagcacccuggcuggcaccaggaaggacgucgaggucaccaaggaggaauucgugcucgccgcccagaaguucgggcaagugacccccauggagguggacauacuguuccagcuggccgaucuguaugagccgcggggcaggaugacccuggccgacauugagcgaaucgccccccuggaggagggcacccugcccuuuaaccuggccgaggcccaaaggcagaaggccagcggggacagcgcaagaccgguccugcugcagguggccgaaagcgccuaccgguucggccugggcagcguggccggagccgucggcgccaccgccguguaccccaucgaccuggugaaaacacggaugcagaaccagaggagcaccggcagcuucgugggcgagcugauguauaagaacagcuuugacugcuucaagaagguccugagguacgagggcuucuucgggcucuacagaggccugcucccccagcuccugggggucgcccccgagaaagcaaucaagcugaccgugaacgacuuugucagggacaaguucaugcacaaggacggcuccgugccccucgccgccgagauccuggccggcggaugcgcggggggaagccaggugaucuuuacgaacccccucgagaucgucaagauuaggcugcagguggccggggagaucaccaccgggcccagggugagcgcccugagcguggugcgcgaucucggcuucuucggcaucuacaagggagccaaggccugcuuccugagggacauccccuucagcgccaucuacuucccguguuacgcccacgugaaggccucguucgccaacgaggacggccaggugagccccgggucgcuccuccuggcgggagccauagccggcaugcccgccgccucccuggugaccccagcggacgugaucaagacccggcuccagguggccgccagggccgggcagaccacguauagcggcgugaucgacugcuuccgaaaaauccugagggaggagggccccaaggcccuguggaaaggcgcgggggccaggguguuccgcuccuccccccaguucggggugacgcugcugacuuacgaguugcugcagaggugguucuacaucgacuuuggcggcgugaagcccauggggagcgagccggugcccaagagccggaucaaccucccagcccccaaccccgaccacgugggcggauacaagcuggccguggccaccuuugccggcaucgaaaacaaguucggccucuaccucccgcuguucaagcccagcguguccacgagcaaggccaucggcgggggcccc

SEQ ID NO: 28 - RNA, 2025 nt, Artificial Sequence
  Citrin-CO24
auggccgccgccaaagucgcccugacaaagcgcgccgaccccgccgagcugcggaccaucuuucugaaguacgccuccaucgagaagaacggcgaguuuuucaugagccccaacgacuucgugacccgcuaccugaacaucuucggcgagagccaaccaaaccccaagaccguggagcugcugucugguguggucgaccagaccaaggauggccugauaucguuccaggaguucguggccuucgagagcguccugugcgcccccgacgcccuguucaugguggccuuccagcuguucgacaaagccggcaagggcgaggugaccuucgaggacgucaaacagguguucggccagaccaccauccaccaacacauaccguucaacugggauuccgaguucguccagcuucauuucgggaaggaaaggaagaggcaccugaccuaugccgaguuuacccaguuccuguuggagauccagcuggagcacgcgaagcaggccuucgugcaacgggacaacgcccggaccgggagggugaccgccaucgacuucagagacauaauggucaccaucaggccgcacgugcucacccccuucguggaggaaugccugguggccgccgccggcgguaccaccucccaccaggucagcuucagcuacuuuaacggcuucaacagccugcugaacaacauggagcugauccgaaagauuuacagcacccuggccggcacgcggaaggacguggaagugaccaaggaggaguuuguacuggccgcccagaaguucggccaggugacgcccauggagguggacaucuuauuccagcuggcggauuuauacgagccccgggggaggaugacccuggccgauaucgagaggaucgccccccuggaagagggcacccugcccuucaaccuugccgaggcccagcggcaaaaagcuagcggcgacagugcaaggcccgugcugcugcagguggcggagagcgccuaccgcuucggccugggcagcguggccggcgccgucggagccaccgccguguaucccaucgaccuggucaagaccaggaugcagaaccagcggagcaccggcagcuucgugggggaacugauguacaagaacagcuuugacugcuucaagaaggugcugagguacgaaggguuuuuugggcuguacagagggcugcugccccagcugcuggguguggcccccgagaaggcaaucaagcugaccgugaacgacuucgugagggacaaguucaugcacaaggacggaucagugccacuggccgccgagauacuggccggcggcugugccgggggcagccaagugaucuucaccaacccccuggagaucgugaagauccgccugcaggucgccggcgagaucaccaccgggccuaggguguccgcccugagcguggugagggaccugggcuucuuugggaucuauaagggcgccaaggccugcuuccugcgcgacaucccauucucugccauauacuuccccugcuacgcccacgugaaagccagcuucgccaacgaagacggccaggugagccccggaagccugcugcuggccggcgccaucgccggaaugcccgccgccucccuggugaccccggccgacgugaucaagaccaggcugcaggucgccgcccgagccgggcagaccaccuauuccggcgugauagacugcuuccgcaagauccuccgagaggaaggucccaaggcccuguggaagggcgccggggcccggguguucaggagcuccccgcaguucggcgugacccugcucaccuacgagcugcugcaaaggugguucuauaucgauuucggcggcgugaagccgaugggcuccgagcccgugcccaagagccggaucaaccugcccgcccccaaccccgaccacguaggcggcuauaagcuggcaguggcaaccuucgccgggaucgaaaacaaauucggccuguaccucccccuguucaaacccagcgugagcacgagcaaggccaucggcggaggcccc

SEQ ID NO: 29 - RNA, 2025 nt, Artificial Sequence
  Citrin-CO25
auggccgccgccaaggucgcccugaccaaaagggccgaccccgccgagcugcgaaccaucuuccugaaauacgccagcauagagaagaacggcgaguucuucaugagcccgaacgacuucgugacgcgguaccugaacaucuucggggagagccagcccaaccccaagaccguggagcugcugagcggcgugguggaucagaccaaggacgggcugaucaguuuccaagaguucguggccuucgagagcgugcugugcgcccccgacgcccuguucaugguggcuuuccagcuguucgacaaggccgggaagggggaggugacauucgaggacgugaagcagguguucgggcagaccacgauccaccagcacauccccuucaacugggacuccgaauuugugcagcugcauuucggcaaggagcggaagaggcaccugaccuacgccgaauucacccaguuccugcuggagauccagcuggaacacgccaagcaggcauucgugcagcgcgacaacgcccgcaccgguagggugaccgccaucgacuuccgggacaucauggugaccauccggccgcacgugcugacccccuucguggaggaaugccugguggccgccgccggcggcaccaccagccaccaagugagcuucagcuauuucaacggcuucaacagccugcucaacaauauggagcugaucaggaaaaucuacagcacccuggccgggaccaggaaggauguggaggugaccaaagaggaauuugugcucgccgcccaaaaguucggccaggucacccccauggaagucgacauccuguuucagcuugccgaccucuaugagcccagggggagaaugacccuggccgacaucgagaggaucgcuccccuggaggagggaacacugccguucaaccuggccgaggcccagaggcagaaggccagcggugacuccgccaggcccguacugcugcaaguggcggaguccgccuauagguucgggcugggcagcguggccggggccgugggggccaccgcgguguacccaauagaccuggugaaaacccggaugcaaaaccagaggagcacggguagcuucgugggggagcugauguauaagaauagcuucgauugcuucaagaagguccuccgguacgagggauucuucggccuguaccggggccugcugccccagcugcugggugucgcccccgagaaggccauaaagcugaccgugaacgauuucgugcgggacaaguucaugcacaaggacggcucggugccccuggccgccgaaauacuggcgggcgggugugccggcgggucccaggugaucuucaccaacccgcuggagaucgugaagauccgucugcagguggccggcgagaucaccaccggccccagaguguccgcgcugagcgucgugcgugaccugggcuucuucgggaucuacaagggagccaaagccugcuuucugagggacauccccuucuccgccaucuacuuccccuguuacgcccacguuaaggccuccuuugccaacgaggacggccaggugagccccgggucccugcugcucgcaggcgccaucgccggcaugcccgccgccagccuggugaccccggccgacgugaucaagacgaggcuccagguggccgccagggcggggcagacuaccuacagcggcguuaucgacugcuuuaggaagauccugagggaggaggggcccaaggcccucuggaagggcgccggagccaggguguucaggagcagcccccaguuugggguaacgcuccugaccuacgagcugcugcagaggugguuuuacaucgauuucgggggcgucaagcccaugggguccgagcccgugcccaagagcaggaucaaucugcccgcccccaaucccgaccacguggggggcuacaagcuggccguggccacguucgccgguaucgagaacaaguucgggcuguaccugccccuguucaagcccuccguauccaccagcaaggcgauaggagggggaccc

SEQ ID NO: 30 - RNA, 47 nt, Artificial Sequence
  (5' UTR)
gggaaauaagagagaaaagaagaguaagaagaaauauaagagccacc

SEQ ID NO: 31 - RNA, 47 nt, Artificial Sequence
  5'UTR-002
gggagaucagagagaaaagaagaguaagaagaaauauaagagccacc

SEQ ID NO: 32 - RNA, 145 nt, Artificial Sequence
  5'UTR-003
ggaauaaaagucucaacacaacauauacaaaacaaacgaaucucaagcaaucaagcauucuacuucuauugcagcaauuuaaaucauuucuuuuaaagcaaaagcaauuuucugaaaauuuucaccauuuacgaacgauagcaac

SEQ ID NO: 33 - RNA, 42 nt, Artificial Sequence
  5'UTR-004
gggagacaagcuuggcauuccgguacuguugguaaagccacc

SEQ ID NO: 34 - RNA, 47 nt, Artificial Sequence; identical to SEQ ID NO: 31
  5'UTR-005

SEQ ID NO: 35 - RNA, 145 nt, Artificial Sequence; identical to SEQ ID NO: 32
  5'UTR-006

SEQ ID NO: 36 - RNA, 42 nt, Artificial Sequence; identical to SEQ ID NO: 33
  5'UTR-007

SEQ ID NO: 37 - RNA, 47 nt, Artificial Sequence
  5'UTR-008
gggaauuaacagagaaaagaagaguaagaagaaauauaagagccacc

SEQ ID NO: 38 - RNA, 47 nt, Artificial Sequence
  5'UTR-009
gggaaauuagacagaaaagaagaguaagaagaaauauaagagccacc

SEQ ID NO: 39 - RNA, 47 nt, Artificial Sequence
  5'UTR-010
gggaaauaagagaguaaagaacaguaagaagaaauauaagagccacc

SEQ ID NO: 40 - RNA, 47 nt, Artificial Sequence
  5'UTR-011
gggaaaaaagagagaaaagaagacuaagaagaaauauaagagccacc

SEQ ID NO: 41 - RNA, 47 nt, Artificial Sequence
  5'UTR-012
gggaaauaagagagaaaagaagaguaagaagauauauaagagccacc

SEQ ID NO: 42 - RNA, 47 nt, Artificial Sequence
  5'UTR-013
gggaaauaagagacaaaacaagaguaagaagaaauauaagagccacc

SEQ ID NO: 43 - RNA, 47 nt, Artificial Sequence
  5'UTR-014
gggaaauuagagaguaaagaacaguaaguagaauuaaaagagccacc

SEQ ID NO: 44 - RNA, 47 nt, Artificial Sequence
  5'UTR-15
gggaaauaagagagaauagaagaguaagaagaaauauaagagccacc

SEQ ID NO: 45 - RNA, 47 nt, Artificial Sequence
  5'UTR-016
gggaaauaagagagaaaagaagaguaagaagaaaauuaagagccacc

SEQ ID NO: 46 - RNA, 47 nt, Artificial Sequence
  5'UTR-017
gggaaauaagagagaaaagaagaguaagaagaaauuuaagagccacc

SEQ ID NO: 47 - RNA, 92 nt, Artificial Sequence
  5'UTR-018
ucaagcuuuuggacccucguacagaagcuaauacgacucacuauagggaaauaagagagaaaagaagaguaagaagaaauauaagagccacc

SEQ ID NO: 48 - RNA, 142 nt, Artificial Sequence
  3'UTR including miR142-3p binding site
ugauaauaguccauaaaguaggaaacacuacagcuggagccucgguggccaugcuucuugccccuugggccuccccccagccccuccuccccuuccugcacccguacccccguggucuuugaauaaagucugagugggcggc

SEQ ID NO: 49 - RNA, 142 nt, Artificial Sequence
  3'UTR including miR142-3p binding site
ugauaauaggcuggagccucgguggcuccauaaaguaggaaacacuacacaugcuucuugccccuugggccuccccccagccccuccuccccuuccugcacccguacccccguggucuuugaauaaagucugagugggcggc

SEQ ID NO: 50 - RNA, 142 nt, Artificial Sequence
  3'UTR including miR142-3p binding site
ugauaauaggcuggagccucgguggccaugcuucuugccccuuccauaaaguaggaaacacuacaugggccuccccccagccccuccuccccuuccugcacccguacccccguggucuuugaauaaagucugagugggcggc

SEQ ID NO: 51 - RNA, 142 nt, Artificial Sequence
  3'UTR including miR142-3p binding site
ugauaauaggcuggagccucgguggccaugcuucuugccccuugggccuccccccaguccauaaaguaggaaacacuacaccccuccuccccuuccugcacccguacccccguggucuuugaauaaagucugagugggcggc

SEQ ID NO: 52 - RNA, 142 nt, Artificial Sequence
  3'UTR including miR142-3p binding site
ugauaauaggcuggagccucgguggccaugcuucuugccccuugggccuccccccagccccuccuccccuucuccauaaaguaggaaacacuacacugcacccguacccccguggucuuugaauaaagucugagugggcggc

SEQ ID NO: 53 - RNA, 142 nt, Artificial Sequence
  3'UTR including miR142-3p binding site
ugauaauaggcuggagccucgguggccaugcuucuugccccuugggccuccccccagccccuccuccccuuccugcacccguacccccuccauaaaguaggaaacacuacaguggucuuugaauaaagucugagugggcggc

SEQ ID NO: 54 - RNA, 142 nt, Artificial Sequence
  3'UTR including miR142-3p binding site
ugauaauaggcuggagccucgguggccaugcuucuugccccuugggccuccccccagccccuccuccccuuccugcacccguacccccguggucuuugaauaaaguuccauaaaguaggaaacacuacacugagugggcggc

SEQ ID NO: 55 - RNA, 371 nt, Artificial Sequence
  3'UTR-001
gcgccugcccaccugccaccgacugcuggaacccagccagugggagggccuggcccaccagaguccugcucccucacuccucgccccgcccccugucccagagucccaccugggggcucucuccacccuucucagaguuccaguuucaaccagaguuccaaccaaugggcuccauccucuggauucuggccaaugaaauaucucccuggcaggguccucuucuuuucccagagcuccaccccaaccaggagcucuaguuaauggagagcucccagcacacucggagcuugugcuuugucuccacgcaaagcgauaaauaaaagcauugguggccuuuggucuuugaauaaagccugaguaggaagucuaga

SEQ ID NO: 56 - RNA, 568 nt, Artificial Sequence
  3'UTR-002
gccccugccgcucccacccccacccaucugggccccggguucaagagagagcggggucugaucucguguagccauauagaguuugcuucugagugucugcuuuguuuaguagaggugggcaggaggagcugaggggcuggggcugggguguugaaguuggcuuugcaugcccagcgaugcgccucccugugggaugucaucacccugggaaccgggaguggcccuuggcucacuguguucugcaugguuuggaucugaauuaauuguccuuucuucuaaaucccaaccgaacuucuuccaaccuccaaacuggcuguaaccccaaauccaagccauuaacuacaccugacaguagcaauugucugauuaaucacuggccccuugaagacagcagaaugucccuuugcaaugaggaggagaucugggcugggcgggccagcuggggaagcauuugacuaucuggaacuugugugugccuccucagguauggcagugacucaccugguuuuaauaaaacaaccugcaacaucucauggucuuugaauaaagccugaguaggaagucuaga

SEQ ID NO: 57 - RNA, 289 nt, Artificial Sequence
  3'UTR-003
acacacuccaccuccagcacgcgacuucucaggacgacgaaucuucucaaugggggggcggcugagcuccagccaccccgcagucacuuucuuuguaacaacuuccguugcugccaucguaaacugacacaguguuuauaacguguacauacauuaacuuauuaccucauuuuguuauuuuucgaaacaaagcccuguggaagaaaauggaaaacuugaagaagcauuaaagucauucuguuaagcugcguaaauggucuuugaauaaagccugaguaggaagucuaga

SEQ ID NO: 58 - RNA, 379 nt, Artificial Sequence
  3'UTR-004
caucacauuuaaaagcaucucagccuaccaugagaauaagagaaagaaaaugaagaucaaaagcuuauucaucuguuuuucuuuuucguugguguaaagccaacacccugucuaaaaaacauaaauuucuuuaaucauuuugccucuuuucucugugcuucaauuaauaaaaaauggaaagaaucuaauagagugguacagcacuguuauuuuucaaagauguguugcuauccugaaaauucuguagguucuguggaaguuccaguguucucucuuauuccacuucgguagaggauuucuaguuucuugugggcuaauuaaauaaaucauuaauacucuucuaauggucuuugaauaaagccugaguaggaagucuaga

SEQ ID NO: 59 - RNA, 118 nt, Artificial Sequence
  3'UTR-005
gcugccuucugcggggcuugccuucuggccaugcccuucuucucucccuugcaccuguaccucuuggucuuugaauaaagccugaguaggaaggcggccgcucgagcaugcaucuaga

SEQ ID NO: 60 - RNA, 908 nt, Artificial Sequence
  3'UTR-006
gccaagcccuccccaucccauguauuuaucucuauuuaauauuuaugucuauuuaagccucauauuuaaagacagggaagagcagaacggagccccaggccucuguguccuucccugcauuucugaguuucauucuccugccuguagcagugagaaaaagcuccuguccucccauccccuggacugggagguagauagguaaauaccaaguauuuauuacuaugacugcuccccagcccuggcucugcaaugggcacugggaugagccgcugugagccccugguccugaggguccccaccugggacccuugagaguaucaggucucccacgugggagacaagaaaucccuguuuaauauuuaaacagcaguguuccccaucuggguccuugcaccccucacucuggccucagccgacugcacagcggccccugcauccccuuggcugugaggccccuggacaagcagagguggccagagcugggaggcauggcccuggggucccacgaauuugcuggggaaucucguuuuucuucuuaagacuuuugggacaugguuugacucccgaacaucaccgacgcgucuccuguuuuucuggguggccucgggacaccugcccugcccccacgagggucaggacugugacucuuuuuagggccaggcaggugccuggacauuugccuugcuggacggggacuggggaugugggagggagcagacaggaggaaucaugucaggccugugugugaaaggaagcuccacugucacccuccaccucuucaccccccacucaccaguguccccuccacugucacauuguaacugaacuucaggauaauaaaguguuugccuccauggucuuugaauaaagccugaguaggaaggcggccgcucgagcaugcaucuaga

SEQ ID NO: 61 - RNA, 835 nt, Artificial Sequence
  3'UTR-007
acucaaucuaaauuaaaaaagaaagaaauuugaaaaaacuuucucuuugccauuucuucuucuucuuuuuuaacugaaagcugaauccuuccauuucuucugcacaucuacuugcuuaaauugugggcaaaagagaaaaagaaggauugaucagagcauugugcaauacaguuucauuaacuccuucccccgcucccccaaaaauuugaauuuuuuuuucaacacucuuacaccuguuauggaaaaugucaaccuuuguaagaaaaccaaaauaaaaauugaaaaauaaaaaccauaaacauuugcaccacuuguggcuuuugaauaucuuccacagagggaaguuuaaaacccaaacuuccaaagguuuaaacuaccucaaaacacuuucccaugagugugauccacauuguuaggugcugaccuagacagagaugaacugagguccuuguuuuguuuuguucauaauacaaaggugcuaauuaauaguauuucagauacuugaagaauguugauggugcuagaagaauuugagaagaaauacuccuguauugaguuguaucgugugguguauuuuuuaaaaaauuugauuuagcauucauauuuuccaucuuauucccaauuaaaaguaugcagauuauuugcccaaaucuucuucagauucagcauuuguucuuugccagucucauuuucaucuucuuccaugguuccacagaagcuuuguuucuugggcaagcagaaaaauuaaauuguaccuauuuuguauaugugagauguuuaaauaaauugugaaaaaaaugaaauaaagcauguuugguuuuccaaaagaacauau

SEQ ID NO: 62 - RNA, 297 nt, Artificial Sequence
  3'UTR-008
cgccgccgcccgggccccgcagucgagggucgugagcccaccccguccauggugcuaagcgggcccgggucccacacggccagcaccgcugcucacucggacgacgcccugggccugcaccucuccagcuccucccacgggguccccguagccccggcccccgcccagccccaggucuccccaggcccuccgcaggcugcccggccucccucccccugcagccaucccaaggcuccugaccuaccuggccccugagcucuggagcaagcccugacccaauaaaggcuuugaacccau

SEQ ID NO: 63 - RNA, 602 nt, Artificial Sequence
  3'UTR-009
ggggcuagagcccucuccgcacagcguggagacggggcaaggagggggguuauuaggauuggugguuuuguuuugcuuuguuuaaagccgugggaaaauggcacaacuuuaccucugugggagaugcaacacugagagccaaggggugggaguugggauaauuuuuauauaaaagaaguuuuuccacuuugaauugcuaaaaguggcauuuuuccuaugugcagucacuccucucauuucuaaaauagggacguggccaggcacgguggcucaugccuguaaucccagcacuuugggaggccgaggcaggcggcucacgaggucaggagaucgagacuauccuggcuaacacgguaaaacccugucucuacuaaaaguacaaaaaauuagcugggcgugguggugggcaccuguagucccagcuacucgggaggcugaggcaggagaaaggcaugaauccaagaggcagagcuugcagugagcugagaucacgccauugcacuccagccugggcaacaguguuaagacucugucucaaauauaaauaaauaaauaaauaaauaaauaaauaaauaaaaauaaagcgagauguugcccucaaa

SEQ ID NO: 64 - RNA, 785 nt, Artificial Sequence
  3'UTR-010
ggcccugccccgucggacugcccccagaaagccuccugcccccugccagugaaguccuucagugagccccuccccagccagcccuucccuggccccgccggauguauaaauguaaaaaugaaggaauuacauuuuauaugugagcgagcaagccggcaagcgagcacaguauuauuucuccauccccucccugccugcuccuuggcacccccaugcugccuucagggagacaggcagggagggcuuggggcugcaccuccuacccucccaccagaacgcaccccacugggagagcugguggugcagccuuccccucccuguauaagacacuuugccaaggcucuccccucucgccccaucccugcuugcccgcucccacagcuuccugagggcuaauucugggaagggagaguucuuugcugccccugucuggaagacguggcucugggugagguaggcgggaaaggauggaguguuuuaguucuugggggaggccaccccaaaccccagccccaacuccaggggcaccuaugagauggccaugcucaaccccccucccagacaggcccucccugucuccagggcccccaccgagguucccagggcuggagacuuccucugguaaacauuccuccagccuccccuccccuggggacgccaaggaggugggccacacccaggaagggaaagcgggcagccccguuuuggggacgugaacguuuuaauaauuuuugcugaauuccuuuacaacuaaauaacacagauauuguuauaaauaaaauugu

SEQ ID NO: 65 - RNA, 3001 nt, Artificial Sequence
  3'UTR-011
auauuaaggaucaagcuguuagcuaauaaugccaccucugcaguuuugggaacaggcaaauaaaguaucaguauacauggugauguacaucuguagcaaagcucuuggagaaaaugaagacugaagaaagcaaagcaaaaacuguauagagagauuuuucaaaagcaguaaucccucaauuuuaaaaaaggauugaaaauucuaaaugucuuucugugcauauuuuuuguguuaggaaucaaaaguauuuuauaaaaggagaaagaacagccucauuuuagauguaguccuguuggauuuuuuaugccuccucaguaaccagaaauguuuuaaaaaacuaaguguuuaggauuucaagacaacauuauacauggcucugaaauaucugacacaauguaaacauugcaggcaccugcauuuuauguuuuuuuuuucaacaaaugugacuaauuugaaacuuuuaugaacuucugagcuguccccuugcaauucaaccgcaguuugaauuaaucauaucaaaucaguuuuaauuuuuuaaauuguacuucagagucuauauuucaagggcacauuuucucacuacuauuuuaauacauuaaaggacuaaauaaucuuucagagaugcuggaaacaaaucauuugcuuuauauguuucauuagaauaccaaugaaacauacaacuugaaaauuaguaauaguauuuuugaagaucccauuucuaauuggagaucucuuuaauuucgaucaacuuauaauguguaguacuauauuaagugcacuugaguggaauucaacauuugacuaauaaaaugaguucaucauguuggcaagugauguggcaauuaucucuggugacaaaagaguaaaaucaaauauuucugccuguuacaaauaucaaggaagaccugcuacuaugaaauagaugacauuaaucugucuucacuguuuauaauacggauggauuuuuuuucaaaucaguguguguuuugaggucuuauguaauugaugacauuugagagaaaugguggcuuuuuuuagcuaccucuuuguucauuuaagcaccaguaaagaucaugucuuuuuauagaaguguagauuuucuuugugacuuugcuaucgugccuaaagcucuaaauauaggugaaugugugaugaauacucagauuauuugucucucuauauaauuaguuugguacuaaguuucucaaaaaauuauuaacacaugaaagacaaucucuaaaccagaaaaagaaguaguacaaauuuuguuacuguaaugcucgcguuuagugaguuuaaaacacacaguaucuuuugguuuuauaaucaguuucuauuuugcugugccugagauuaagaucuguguaugugugugugugugugugugcguuuguguguuaaagcagaaaagacuuuuuuaaaaguuuuaagugauaaaugcaauuuguuaauugaucuuagaucacuaguaaacucagggcugaauuauaccauguauauucuauuagaagaaaguaaacaccaucuuuauuccugcccuuuuucuucucucaaaguaguuguaguuauaucuagaaagaagcaauuuugauuucuugaaaagguaguuccugcacucaguuuaaacuaaaaauaaucauacuuggauuuuauuuauuuuugucauaguaaaaauuuuaauuuauauauauuuuuauuuaguauuaucuuauucuuugcuauuugccaauccuuugucaucaauuguguuaaaugaauugaaaauucaugcccuguucauuuuauuuuacuuuauugguuaggauauuuaaaggauuuuuguauauauaauuucuuaaauuaauauuccaaaagguuaguggacuuagauuauaaauuauggcaaaaaucuaaaaacaacaaaaaugauuuuuauacauucuauuucauuauuccucuuuuuccaauaagucauacaauugguagauaugacuuauuuuauuuuuguauuauucacuauaucuuuaugauauuuaaguauaaauaauuaaaaaaauuuauuguaccuuauagucugucaccaaaaaaaaaaaauuaucuguagguagugaaaugcuaauguugauuugucuuuaagggcuuguuaacuauccuuuauuuucucauuugucuuaaauuaggaguuuguguuuaaauuacucaucuaagcaaaaaauguauauaaaucccauuacuggguauauacccaaaggauuauaaaucaugcugcuauaaagacacaugcacacguauguuuauugcagcacuauucacaauagcaaagacuuggaaccaacccaaauguccaucaaugauagacuugauuaagaaaaugugcacauauacaccauggaauacuaugcagccauaaaaaaggaugaguucauguccuuuguagggacauggauaaagcuggaaaccaucauucugagcaaacuauugcaaggacagaaaaccaaacacugcauguucucacucauaggugggaauugaacaaugagaacacuuggacacaagguggggaacaccacacaccagggccugucaugggguggggggaguggggagggauagcauuaggagauauaccuaauguaaaugaugaguuaaugggugcagcacaccaacauggcacauguauacauauguagcaaaccugcacguugugcacauguacccuagaacuuaaaguauaauuaaaaaaaaaaagaaaacagaagcuauuuauaaagaaguuauuugcugaaauaaaugugaucuuucccauuaaaaaaauaaagaaauuuugggguaaaaaaacacaauauauuguauucuugaaaaauucuaagagaguggaugugaaguguucucaccacaaaagugauaacuaauugagguaaugcacauauuaauuagaaagauuuugucauuccacaauguauauauacuuaaaaauauguuauacacaauaaauacauacauuaaaaaauaaguaaaugua

SEQ ID NO: 66 - RNA, 1037 nt, Artificial Sequence
  3'UTR-012
cccacccugcacgccggcaccaaacccuguccucccaccccuccccacucaucacuaaacagaguaaaaugugaugcgaauuuucccgaccaaccugauucgcuagauuuuuuuuaaggaaaagcuuggaaagccaggacacaacgcugcugccugcuuugugcaggguccuccggggcucagcccugaguuggcaucaccugcgcagggcccucuggggcucagcccugagcuagugucaccugcacagggcccucugaggcucagcccugagcuggcgucaccugugcagggcccucuggggcucagcccugagcuggccucaccuggguuccccaccccgggcucuccugcccugcccuccugcccgcccucccuccugccugcgcagcuccuucccuaggcaccucugugcugcaucccaccagccugagcaagacgcccucucggggccugugccgcacuagccucccucuccucuguccccauagcugguuuuucccaccaauccucaccuaacaguuacuuuacaauuaaacucaaagcaagcucuucuccucagcuuggggcagccauuggccucugucucguuuugggaaaccaaggucaggaggccguugcagacauaaaucucggcgacucggccccgucuccugaggguccugcuggugaccggccuggaccuuggcccuacagcccuggaggccgcugcugaccagcacugaccccgaccucagagaguacucgcaggggcgcuggcugcacucaagacccucgagauuaacggugcuaaccccgucugcuccucccucccgcagagacuggggccuggacuggacaugagagccccuuggugccacagagggcugugucuuacuagaaacaacgcaaaccucuccuuccucagaauagugauguguucgacguuuuaucaaaggcccccuuucuauguucauguuaguuuugcuccuucuguguuuuuuucugaaccauauccauguugcugacuuuuccaaauaaagguuuucacuccucuc

SEQ ID NO: 67 - RNA, 577 nt, Artificial Sequence
  3'UTR-013
agaggccugccuccagggcuggacugaggccugagcgcuccugccgcagagcuggccgcgccaaauaaugucucugugagacucgagaacuuucauuuuuuuccaggcugguucggauuugggguggauuuugguuuuguuccccuccuccacucucccccacccccuccccgcccuuuuuuuuuuuuuuuuuuaaacugguauuuuaucuuugauucuccuucagcccucaccccugguucucaucuuucuugaucaacaucuuuucuugccucuguccccuucucucaucucuuagcuccccuccaaccuggggggcagugguguggagaagccacaggccugagauuucaucugcucuccuuccuggagcccagaggagggcagcagaaggggguggugucuccaaccccccagcacugaggaagaacggggcucuucucauuucaccccucccuuucuccccugcccccaggacugggccacuucuggguggggcagugggucccagauuggcucacacugagaauguaagaacuacaaacaaaauuucuauuaaauuaaauuuugugucucc

SEQ ID NO: 68 - RNA, 2212 nt, Artificial Sequence
  3'UTR-014
cucccuccaucccaaccuggcucccucccacccaaccaacuuuccccccaacccggaaacagacaagcaacccaaacugaacccccucaaaagccaaaaaaugggagacaauuucacauggacuuuggaaaauauuuuuuuccuuugcauucaucucucaaacuuaguuuuuaucuuugaccaaccgaacaugaccaaaaaccaaaagugcauucaaccuuaccaaaaaaaaaaaaaaaaaaagaauaaauaaauaacuuuuuaaaaaaggaagcuugguccacuugcuugaagacccaugcggggguaagucccuuucugcccguugggcuuaugaaaccccaaugcugcccuuucugcuccuuucuccacaccccccuuggggccuccccuccacuccuucccaaaucugucuccccagaagacacaggaaacaauguauugucugcccagcaaucaaaggcaaugcucaaacacccaaguggcccccacccucagcccgcuccugcccgcccagcacccccaggcccugggggaccugggguucucagacugccaaagaagccuugccaucuggcgcucccauggcucuugcaacaucuccccuucguuuuugagggggucaugccgggggagccaccagccccucacuggguucggaggagagucaggaagggccacgacaaagcagaaacaucggauuuggggaacgcgugucaaucccuugugccgcagggcugggcgggagagacuguucuguuccuuguguaacuguguugcugaaagacuaccucguucuugucuugaugugucaccggggcaacugccugggggcggggaugggggcaggguggaagcggcuccccauuuuauaccaaaggugcuacaucuaugugaugggugggguggggagggaaucacuggugcuauagaaauugagaugcccccccaggccagcaaauguuccuuuuuguucaaagucuauuuuuauuccuugauauuuuucuuuuuuuuuuuuuuuuuuuguggauggggacuugugaauuuuucuaaaggugcuauuuaacaugggaggagagcgugugcggcuccagcccagcccgcugcucacuuuccacccucucuccaccugccucuggcuucucaggccucugcucuccgaccucucuccucugaaacccuccuccacagcugcagcccauccucccggcucccuccuagucuguccugcguccucuguccccggguuucagagacaacuucccaaagcacaaagcaguuuuucccccuaggggugggaggaagcaaaagacucuguaccuauuuuguauguguauaauaauuugagauguuuuuaauuauuuugauugcuggaauaaagcauguggaaaugacccaaacauaauccgcaguggccuccuaauuuccuucuuuggaguugggggagggguagacauggggaaggggcuuuggggugaugggcuugccuuccauuccugcccuuucccuccccacuauucucuucuagaucccuccauaaccccacuccccuuucucucacccuucuuauaccgcaaaccuuucuacuuccucuuucauuuucuauucuugcaauuuccuugcaccuuuuccaaauccucuucuccccugcaauaccauacaggcaauccacgugcacaacacacacacacacucuucacaucugggguuguccaaaccucauacccacuccccuucaagcccauccacucuccacccccuggaugcccugcacuugguggcggugggaugcucauggauacugggagggugaggggaguggaacccgugaggaggaccugggggccucuccuugaacugacaugaagggucaucuggccucugcucccuucucacccacgcugaccuccugccgaaggagcaacgcaacaggagaggggucugcugagccuggcgagggucugggagggaccaggaggaaggcgugcucccugcucgcuguccuggcccugggggagugagggagacagacaccugggagagcuguggggaaggcacucgcaccgugcucuugggaaggaaggagaccuggcccugcucaccacggacugggugccucgaccuccugaauccccagaacacaaccccccugggcugggguggucuggggaaccaucgugcccccgccucccgccuacuccuuuuuaagcuu

SEQ ID NO: 69 - RNA, 729 nt, Artificial Sequence
  3'UTR-015
uuggccaggccugacccucuuggaccuuucuucuuugccgacaaccacugcccagcagccucugggaccucggggucccagggaacccaguccagccuccuggcuguugacuucccauugcucuuggagccaccaaucaaagagauucaaagagauuccugcaggccagaggcggaacacaccuuuauggcuggggcucuccgugguguucuggacccagccccuggagacaccauucacuuuuacugcuuuguagugacucgugcucuccaaccugucuuccugaaaaaccaaggcccccuucccccaccucuuccauggggugagacuugagcagaacaggggcuuccccaaguugcccagaaagacugucugggugagaagccauggccagagcuucucccaggcacagguguugcaccagggacuucugcuucaaguuuugggguaaagacaccuggaucagacuccaagggcugcccugagucugggacuucugccuccauggcuggucaugagagcaaaccguaguccccuggagacagcgacuccagagaaccucuugggagacagaagaggcaucugugcacagcucgaucuucuacuugccuguggggaggggagugacagguccacacaccacacugggucacccuguccuggaugccucugaagagagggacagaccgucagaaacuggagaguuucuauuaaaggucauuuaaacca

SEQ ID NO: 70 - RNA, 847 nt, Artificial Sequence
  3'UTR-016
uccuccgggaccccagcccucaggauuccugaugcuccaaggcgacugaugggcgcuggaugaaguggcacagucagcuucccugggggcuggugucauguugggcuccuggggcgggggcacggccuggcauuucacgcauugcugccaccccagguccaccugucuccacuuucacagccuccaagucuguggcucuucccuucuguccuccgaggggcuugccuucucucguguccagugaggugcucagugaucggcuuaacuuagagaagcccgcccccuccccuucuccgucugucccaagagggucugcucugagccugcguuccuagguggcucggccucagcugccuggguuguggccgcccuagcauccuguaugcccacagcuacuggaauccccgcugcugcuccgggccaagcuucugguugauuaaugagggcaugggguggucccucaagaccuuccccuaccuuuuguggaaccagugaugccucaaagacaguguccccuccacagcugggugccaggggcaggggauccucaguauagccggugaacccugauaccaggagccugggccucccugaaccccuggcuuccagccaucucaucgccagccuccuccuggaccucuuggcccccagccccuuccccacacagccccagaagggucccagagcugaccccacuccaggaccuaggcccagccccucagccucaucuggagccccugaagaccagucccacccaccuuucuggccucaucugacacugcuccgcauccugcuguguguccuguuccauguuccgguuccauccaaauacacuuucuggaacaaa

SEQ ID NO: 71 - RNA, 110 nt, Artificial Sequence
  3'UTR-017
gcuggagccucgguggccaugcuucuugccccuugggccuccccccagccccuccuccccuuccugcacccguacccccguggucuuugaauaaagucugagugggcggc

SEQ ID NO: 72 - RNA, 119 nt, Artificial Sequence
  3' UTR no miR binding sites
ugauaauaggcuggagccucgguggccaugcuucuugccccuugggccuccccccagccccuccuccccuuccugcacccguacccccguggucuuugaauaaagucugagugggcggc

SEQ ID NO: 73 - RNA, 87 nt, Artificial Sequence
  miR-142
gacagugcagucacccauaaaguagaaagcacuacuaacagcacuggaggguguaguguuuccuacuuuauggaugaguguacugug

SEQ ID NO: 74 - RNA, 23 nt, Artificial Sequence
  miR-142-3p
uguaguguuuccuacuuuaugga

SEQ ID NO: 75 - RNA, 23 nt, Artificial Sequence
  miR-142-3p binding site
uccauaaaguaggaaacacuaca

SEQ ID NO: 76 - RNA, 21 nt, Artificial Sequence
  miR-142-5p
cauaaaguagaaagcacuacu

SEQ ID NO: 77 - RNA, 21 nt, Artificial Sequence
  miR-142-5p binding site
aguagugcuuucuacuuuaug

SEQ ID NO: 78 - DNA, 18 bp, Artificial Sequence
  Syn5 promoter
attgggcacccgtaaggg

SEQ ID NO: 79 - RNA, 92 nt, Artificial Sequence; identical to SEQ ID NO: 47
  5' UTR of Citrin in Example 12

SEQ ID NO: 80 - RNA, 119 nt, Artificial Sequence; identical to SEQ ID NO: 72
  3' UTR of Citrin in Example 12

SEQ ID NO: 81 - RNA, 133 nt, Artificial Sequence
  (3'UTR with miR 142-3p binding site)
gcuggagccucgguggccaugcuucuugccccuugggccuccccccagccccuccuccccuuccugcacccguacccccuccauaaaguaggaaacacuacaguggucuuugaauaaagucugagugggcggc

SEQ ID NO: 82 - RNA, 23 nt, Artificial Sequence
  (miR 142-3p binding site)
uccauaaaguaggaaacacuaca

SEQ ID NO: 83 - RNA, 23 nt, Artificial Sequence
  (miR 142-3p sequence)
uguaguguuuccuacuuuaugga

SEQ ID NO: 84 - RNA, 21 nt, Artificial Sequence
  (miR 142-5p sequence)
cauaaaguagaaagcacuacu

SEQ ID NO: 85 - RNA, 22 nt, Artificial Sequence
  (miR 146-3p sequence)
ccucugaaauucaguucuucag

SEQ ID NO: 86 - RNA, 22 nt, Artificial Sequence
  (miR 146-5p sequence)
ugagaacugaauuccauggguu

SEQ ID NO: 87 - RNA, 22 nt, Artificial Sequence
  (miR 155-3p sequence)
cuccuacauauuagcauuaaca

SEQ ID NO: 88 - RNA, 23 nt, Artificial Sequence
  (miR 155-5p sequence)
uuaaugcuaaucgugauaggggu

SEQ ID NO: 89 - RNA, 22 nt, Artificial Sequence
  (miR 126-3p sequence)
ucguaccgugaguaauaaugcg

SEQ ID NO: 90 - RNA, 21 nt, Artificial Sequence
  (miR 126-5p sequence)
cauuauuacuuuugguacgcg

SEQ ID NO: 91 - RNA, 22 nt, Artificial Sequence
  (miR 16-3p sequence)
ccaguauuaacugugcugcuga

SEQ ID NO: 92 - RNA, 22 nt, Artificial Sequence
  (miR 16-5p sequence)
uagcagcacguaaauauuggcg

SEQ ID NO: 93 - RNA, 21 nt, Artificial Sequence
  (miR 21-3p sequence)
caacaccagucgaugggcugu

SEQ ID NO: 94 - RNA, 22 nt, Artificial Sequence
  (miR 21-5p sequence)
uagcuuaucagacugauguuga

SEQ ID NO: 95 - RNA, 22 nt, Artificial Sequence
  (miR 223-3p sequence)
ugucaguuugucaaauacccca

SEQ ID NO: 96 - RNA, 22 nt, Artificial Sequence
  (miR 223-5p sequence)
cguguauuugacaagcugaguu

SEQ ID NO: 97 - RNA, 22 nt, Artificial Sequence
  (miR 24-3p sequence)
uggcucaguucagcaggaacag

SEQ ID NO: 98 - RNA, 22 nt, Artificial Sequence
  (miR 24-5p sequence)
ugccuacugagcugauaucagu

SEQ ID NO: 99 - RNA, 21 nt, Artificial Sequence
  (miR 27-3p sequence)
uucacaguggcuaaguuccgc

SEQ ID NO: 100 - RNA, 22 nt, Artificial Sequence
  (miR 27-5p sequence)
agggcuuagcugcuugugagca

SEQ ID NO: 101 - RNA, 22 nt, Artificial Sequence
  (miR 126-3p binding site)
cgcauuauuacucacgguacga

SEQ ID NO: 102 - RNA, 141 nt, Artificial Sequence
  (3'UTR with miR 126-3p binding site)
ugauaauaggcuggagccucgguggccaugcuucuugccccuugggccuccccccagccccuccuccccuuccugcacccguaccccccgcauuauuacucacgguacgaguggucuuugaauaaagucugagugggcggc

SEQ ID NO: 103 - RNA, 142 nt, Artificial Sequence; identical to SEQ ID NO: 53
  (3' UTR with miR 142-3p binding site)

SEQ ID NO: 104 - RNA, 141 nt, Artificial Sequence; identical to SEQ ID NO: 102
  (3' UTR with miR 126-3p binding site)

SEQ ID NO: 105 - RNA, 164 nt, Artificial Sequence
  (3' UTR with miR 142-3p and miR 126-3p binding sites)
ugauaauaguccauaaaguaggaaacacuacagcuggagccucgguggccaugcuucuugccccuugggccuccccccagccccuccuccccuuccugcacccguaccccccgcauuauuacucacgguacgaguggucuuugaauaaagucugagugggcggc

SEQ ID NO: 106 - RNA, 23 nt, Artificial Sequence
  (miR 155-5p sequence)
uuaaugcuaauugugauaggggu

SEQ ID NO: 107 - RNA, 23 nt, Artificial Sequence
  (miR 155-5p binding site)
accccuaucacaauuagcauuaa

SEQ ID NO: 108 - RNA, 188 nt, Artificial Sequence
  (3' UTR with 3 miR 142-3p binding sites)
ugauaauaguccauaaaguaggaaacacuacagcuggagccucgguggccaugcuucuugccccuugggccuccauaaaguaggaaacacuacauccccccagccccuccuccccuuccugcacccguacccccuccauaaaguaggaaacacuacaguggucuuugaauaaagucugagugggcggc

SEQ ID NO: 109 - RNA, 140 nt, Artificial Sequence
  (3'UTR with miR 142-5p binding site)
ugauaauaggcuggagccucgguggccaugcuucuugccccuugggccuccccccagccccuccuccccuuccugcacccguacccccaguagugcuuucuacuuuaugguggucuuugaauaaagucugagugggcggc

SEQ ID NO: 110 - RNA, 182 nt, Artificial Sequence
  (3'UTR with 3 miR 142-5p binding sites)
ugauaauagaguagugcuuucuacuuuauggcuggagccucgguggccaugcuucuugccccuugggccaguagugcuuucuacuuuauguccccccagccccuccuccccuuccugcacccguacccccaguagugcuuucuacuuuaugguggucuuugaauaaagucugagugggcggc

SEQ ID NO: 111 - RNA, 184 nt, Artificial Sequence
  (3'UTR with 2 miR 142-5p binding sites and 1 miR 142-3p binding site)
ugauaauagaguagugcuuucuacuuuauggcuggagccucgguggccaugcuucuugccccuugggccuccauaaaguaggaaacacuacauccccccagccccuccuccccuuccugcacccguacccccaguagugcuuucuacuuuaugguggucuuugaauaaagucugagugggcggc

SEQ ID NO: 112 - RNA, 142 nt, Artificial Sequence
  (3'UTR with miR 155-5p binding site)
ugauaauaggcuggagccucgguggccaugcuucuugccccuugggccuccccccagccccuccuccccuuccugcacccguacccccaccccuaucacaauuagcauuaaguggucuuugaauaaagucugagugggcggc

SEQ ID NO: 113 - RNA, 188 nt, Artificial Sequence
  (3' UTR with 3 miR 155-5p binding sites)
ugauaauagaccccuaucacaauuagcauuaagcuggagccucgguggccaugcuucuugccccuugggccaccccuaucacaauuagcauuaauccccccagccccuccuccccuuccugcacccguacccccaccccuaucacaauuagcauuaaguggucuuugaauaaagucugagugggcggc

SEQ ID NO: 114 - RNA, 188 nt, Artificial Sequence
  (3'UTR with 2 miR 155-5p binding sites and 1 miR 142-3p binding site)
ugauaauagaccccuaucacaauuagcauuaagcuggagccucgguggccaugcuucuugccccuugggccuccauaaaguaggaaacacuacauccccccagccccuccuccccuuccugcacccguacccccaccccuaucacaauuagcauuaaguggucuuugaauaaagucugagugggcggc

SEQ ID NO: 115 - RNA, 142 nt, Artificial Sequence; identical to SEQ ID NO: 48
  (3'UTR with miR 142-3p binding site, P1 insertion)

SEQ ID NO: 116 - RNA, 142 nt, Artificial Sequence; identical to SEQ ID NO: 49
  (3'UTR with miR 142-3p binding site, P2 insertion)

SEQ ID NO: 117 - RNA, 142 nt, Artificial Sequence
  (3'UTR with miR 142-3p binding site, P3 insertion)
ugauaauaggcuggagccucgguggccaugcuucuugccccuugggccuccauaaaguaggaaacacuacauccccccagccccuccuccccuuccugcacccguacccccguggucuuugaauaaagucugagugggcggc

SEQ ID NO: 118 - RNA, 21 nt, Artificial Sequence
  (miR-142-5p binding site)
aguagugcuuucuacuuuaug

SEQ ID NO: 119 - RNA, 87 nt, Artificial Sequence; identical to SEQ ID NO: 73
  (miR-142)

SEQ ID NO: 120 - RNA, 70 nt, Artificial Sequence
  (5' UTR with miR142-3p binding site at position p1)
gggaaauaagaguccauaaaguaggaaacacuacaagaaaagaagaguaagaagaaauauaagagccacc

SEQ ID NO: 121 - RNA, 70 nt, Artificial Sequence
  (5' UTR with miR142-3p binding site at position p2)
gggaaauaagagagaaaagaagaguaauccauaaaguaggaaacacuacagaagaaauauaagagccacc

SEQ ID NO: 122 - RNA, 70 nt, Artificial Sequence
  (5' UTR with miR142-3p binding site at position p3)
gggaaauaagagagaaaagaagaguaagaagaaauauaauccauaaaguaggaaacacuacagagccacc

SEQ ID NO: 123 - RNA, 23 nt, Artificial Sequence
  (miR 155-5p binding site)
accccuaucacaauuagcauuaa

SEQ ID NO: 124 - RNA, 181 nt, Artificial Sequence
  (3'UTR with 3 miR 142-5p binding sites)
ugauaauagaguagugcuuucuacuuuauggcuggagccucgguggccaugcuucuugccccuugggccaguagugcuuucuacuuuauguccccccagccccucuccccuuccugcacccguacccccaguagugcuuucuacuuuaugguggucuuugaauaaagucugagugggcggc

SEQ ID NO: 125 - RNA, 184 nt, Artificial Sequence; identical to SEQ ID NO: 111
  (3'UTR with 2 miR 142-5p binding sites and 1 miR 142-3p binding site)

SEQ ID NO: 126 - RNA, 70 nt, Artificial Sequence; identical to SEQ ID NO: 120
  (5' UTR with miR142-3p binding site at position p1)

SEQ ID NO: 127 - RNA, 70 nt, Artificial Sequence; identical to SEQ ID NO: 121
  (5' UTR with miR142-3p binding site at position p2)

SEQ ID NO: 128 - RNA, 70 nt, Artificial Sequence; identical to SEQ ID NO: 122
  (5' UTR with miR142-3p binding site at position p3)

SEQ ID NO: 129 - RNA, 2025 nt, Artificial Sequence
  Construct #1 ORF of Citrin gene
auggccgccgccaaggucgcccucaccaagagggcggaccccgcggagcucaggaccaucuuucucaaguacgccuccaucgagaagaacggggaguucuucaugagcccgaacgauuucgucaccagguaccucaacaucuucggcgagagccagcccaacccgaagaccguagagcuccucagcggcgucgucgaccagacgaaggacggacucauuagcuuccaggaguucgucgccuucgagagcguccucugcgcgcccgacgcccucuucauggucgcguuccagcuguucgauaaggccggcaagggcgaggugaccuuugaagaugugaagcagguguucggucagaccaccauccaccagcacaucccuuuuaacugggacucagaauucguccagcugcacuucggcaaggaaaggaagcgccaucugaccuacgccgaguucacacaguuucuccuggagauccagcuggaacacgccaaacaggcguucguucagcgggacaacgccaggaccggccgggucaccgcgaucgacuuccgugauaucauggugaccaucaggccucacguccugacgcccuucguggaagagugccugguggccgccgcgggugggaccacgucccaccaggugagcuucuccuauuuuaacggguucaacagccuccucaacaacauggagcugauccggaagaucuauagcacccuggccgggacgcgcaaggacgucgaggugaccaaggaagaauucgugcuggccgcccagaaguuuggccaggugacgcccauggagguggacauccuguuccaacuggcggaccuguacgaacccaggggccggaugacccuggccgacaucgagcgcauugccccgcucgaggagggcacccugcccuucaaccuggcggaggcccagcgccagaaggccagcggggacagcgccaggcccguccugcugcagguggccgaguccgcguacagguucggucuggggagcgucgcgggagccgugggugccaccgccguguauccgaucgaccucgugaagacccguaugcagaaucagagguccaccggcagcuucgugggcgagcucauguacaagaacuccuucgacuguuucaagaagguucuccgguacgagggguucuucggccucuaccggggacugcuaccccagcugcucggcguggcgcccgagaaggccaucaagcucacggucaacgacuuugugcgggacaaguucaugcacaaggacggcagcgucccacuggccgccgagauucuggcaggcggcugcgccggaggcagccaggucaucuuuaccaacccacuggagaucgugaagaucaggcugcaaguggccggggagauuaccaccggaccccgugugagcgcccugagcguggugagggaccuuggcuucuuuggcauauacaagggagccaaggccugcuuucugagggacaucccguuuuccgccauauacuuucccugcuacgcccacgugaaagcgagcuucgccaacgaggacggccaggucagucccggcucccuacugcuggccggagccaucgccgggaugcccgccgccagccuggugacgcccgcggacguuaucaagaccaggcugcagguggcggccagggcgggccagaccaccuacagcggcgugaucgacugcuuccgcaagauccugcgggaggaggggcccaaggcccuguggaaaggcgccggggcaaggguguucaggagcagcccacaguucggggugacccugcuuaccuacgaacugcugcagcggugguucuauaucgacuucggaggagucaagcccaugggcuccgagccugugcccaagagcaggaucaaucugcccgcgcccaacccagaccacgugggaggguacaaacuggccguggccaccuucgccggaaucgagaacaaguucggccuguaucugccccuguucaaaccguccgucuccaccagcaaggccaucggcggaggcccc

SEQ ID NO: 130 - RNA, 2236 nt, Artificial Sequence
  Construct #1 Full Citrin nucleic acid with UTRs
gggaaauaagagagaaaagaagaguaagaagaaauauaagagccaccauggccgccgccaaggucgcccucaccaagagggcggaccccgcggagcucaggaccaucuuucucaaguacgccuccaucgagaagaacggggaguucuucaugagcccgaacgauuucgucaccagguaccucaacaucuucggcgagagccagcccaacccgaagaccguagagcuccucagcggcgucgucgaccagacgaaggacggacucauuagcuuccaggaguucgucgccuucgagagcguccucugcgcgcccgacgcccucuucauggucgcguuccagcuguucgauaaggccggcaagggcgaggugaccuuugaagaugugaagcagguguucggucagaccaccauccaccagcacaucccuuuuaacugggacucagaauucguccagcugcacuucggcaaggaaaggaagcgccaucugaccuacgccgaguucacacaguuucuccuggagauccagcuggaacacgccaaacaggcguucguucagcgggacaacgccaggaccggccgggucaccgcgaucgacuuccgugauaucauggugaccaucaggccucacguccugacgcccuucguggaagagugccugguggccgccgcgggugggaccacgucccaccaggugagcuucuccuauuuuaacggguucaacagccuccucaacaacauggagcugauccggaagaucuauagcacccuggccgggacgcgcaaggacgucgaggugaccaaggaagaauucgugcuggccgcccagaaguuuggccaggugacgcccauggagguggacauccuguuccaacuggcggaccuguacgaacccaggggccggaugacccuggccgacaucgagcgcauugccccgcucgaggagggcacccugcccuucaaccuggcggaggcccagcgccagaaggccagcggggacagcgccaggcccguccugcugcagguggccgaguccgcguacagguucggucuggggagcgucgcgggagccgugggugccaccgccguguauccgaucgaccucgugaagacccguaugcagaaucagagguccaccggcagcuucgugggcgagcucauguacaagaacuccuucgacuguuucaagaagguucuccgguacgagggguucuucggccucuaccggggacugcuaccccagcugcucggcguggcgcccgagaaggccaucaagcucacggucaacgacuuugugcgggacaaguucaugcacaaggacggcagcgucccacuggccgccgagauucuggcaggcggcugcgccggaggcagccaggucaucuuuaccaacccacuggagaucgugaagaucaggcugcaaguggccggggagauuaccaccggaccccgugugagcgcccugagcguggugagggaccuuggcuucuuuggcauauacaagggagccaaggccugcuuucugagggacaucccguuuuccgccauauacuuucccugcuacgcccacgugaaagcgagcuucgccaacgaggacggccaggucagucccggcucccuacugcuggccggagccaucgccgggaugcccgccgccagccuggugacgcccgcggacguuaucaagaccaggcugcagguggcggccagggcgggccagaccaccuacagcggcgugaucgacugcuuccgcaagauccugcgggaggaggggcccaaggcccuguggaaaggcgccggggcaaggguguucaggagcagcccacaguucggggugacccugcuuaccuacgaacugcugcagcggugguucuauaucgacuucggaggagucaagcccaugggcuccgagccugugcccaagagcaggaucaaucugcccgcgcccaacccagaccacgugggaggguacaaacuggccguggccaccuucgccggaaucgagaacaaguucggccuguaucugccccuguucaaaccguccgucuccaccagcaaggccaucggcggaggccccugauaauaguccauaaaguaggaaacacuacagcuggagccucgguggccaugcuucuugccccuugggccuccccccagccccuccuccccuuccugcacccguaccccccgcauuauuacucacgguacgaguggucuuugaauaaagucugagugggcggc

SEQ ID NO: 131 - protein, 675 aa, Artificial Sequence; identical to SEQ ID NO: 1
  Construct #1 Amino acid sequence of Citrin gene

SEQ ID NO: 132 - RNA, 2025 nt, Artificial Sequence
  Construct #2 ORF of Citrin gene
auggccgccgccaaggucgcccucaccaagagggcggaccccgcggagcucaggaccaucuuucucaaguacgccuccaucgagaagaacggggaguucuucaugagcccgaacgauuucgucaccagguaccucaacaucuucggcgagagccagcccaacccgaagaccguagagcuccucagcggcgucgucgaccagacgaaggacggacucauuagcuuccaggaguucgucgccuucgagagcguccucugcgcccccgacgcccucuucauggucgcguuccagcuguucgauaaggccggcaagggcgaggugaccuuugaagaugugaagcagguguucggucagaccaccauccaccagcacaucccuuuuaacugggacucagaauucguccagcugcacuucggcaaggaaaggaagcgccaucugaccuacgccgaguucacacaguuucuccuggagauccagcuggaacacgccaaacaggcguucguucagcgggacaacgccaggaccggccgggucaccgcgaucgacuuccgugauaucauggugaccaucaggccucacguccugacccccuucguggaagagugccugguggccgccgcgggugggaccacgucccaccaggugagcuucuccuauuuuaacggguucaacagccuccucaacaacauggagcugauccggaagaucuauagcacccuggccgggacgcgcaaggacgucgaggugaccaaggaagaauucgugcuggccgcccagaaguuuggccaggugacccccauggagguggacauccuguuccaacuggcggaccuguacgaacccaggggccggaugacccuggccgacaucgagcgcauugccccgcucgaggagggcacccugcccuucaaccuggcggaggcccagcgccagaaggccagcggggacagcgccaggcccguccugcugcagguggccgaguccgcguacagguucggucuggggagcgucgcgggagccgugggugccaccgccguguauccgaucgaccucgugaagacccguaugcagaaucagagguccaccggcagcuucgugggcgagcucauguacaagaacuccuucgacuguuucaagaagguucuccgguacgagggguucuucggccucuaccgggggcugcuaccccagcugcucggcguggcgcccgagaaggccaucaagcucacggucaacgacuuugugcgggacaaguucaugcacaaggacggcagcgucccccuggccgccgagauucuggcaggcggcugcgccggaggcagccaggucaucuuuaccaacccccuggagaucgugaagaucaggcugcaaguggccggggagauuaccaccggaccccgugugagcgcccugagcguggugagggaccuuggcuucuuuggcauauacaagggagccaaggccugcuuucugagggacaucccguuuuccgccauauacuuucccugcuacgcccacgugaaagcgagcuucgccaacgaggacggccaggucagucccggcucccuacugcuggccggagccaucgccgggaugcccgccgccagccuggugacccccgcggacguuaucaagaccaggcugcagguggcggccagggcgggccagaccaccuacagcggcgugaucgacugcuuccgcaagauccugcgggaggaggggcccaaggcccuguggaaaggcgccggggcaaggguguucaggagcagcccccaguucggggugacccugcuuaccuacgaacugcugcagcggugguucuauaucgacuucgggggagucaagcccaugggcuccgagccugugcccaagagcaggaucaaucugcccgcccccaacccagaccacgugggaggguacaaacuggccguggccaccuucgccggaaucgagaacaaguucggccuguaucugccccuguucaaaccguccgucuccaccagcaaggccaucggcgggggcccc

SEQ ID NO: 133 - RNA, 2236 nt, Artificial Sequence
  Construct #2 Full Citrin nucleic acid with UTRs
gggaaauaagagagaaaagaagaguaagaagaaauauaagagccaccauggccgccgccaaggucgcccucaccaagagggcggaccccgcggagcucaggaccaucuuucucaaguacgccuccaucgagaagaacggggaguucuucaugagcccgaacgauuucgucaccagguaccucaacaucuucggcgagagccagcccaacccgaagaccguagagcuccucagcggcgucgucgaccagacgaaggacggacucauuagcuuccaggaguucgucgccuucgagagcguccucugcgcccccgacgcccucuucauggucgcguuccagcuguucgauaaggccggcaagggcgaggugaccuuugaagaugugaagcagguguucggucagaccaccauccaccagcacaucccuuuuaacugggacucagaauucguccagcugcacuucggcaaggaaaggaagcgccaucugaccuacgccgaguucacacaguuucuccuggagauccagcuggaacacgccaaacaggcguucguucagcgggacaacgccaggaccggccgggucaccgcgaucgacuuccgugauaucauggugaccaucaggccucacguccugacccccuucguggaagagugccugguggccgccgcgggugggaccacgucccaccaggugagcuucuccuauuuuaacggguucaacagccuccucaacaacauggagcugauccggaagaucuauagcacccuggccgggacgcgcaaggacgucgaggugaccaaggaagaauucgugcuggccgcccagaaguuuggccaggugacccccauggagguggacauccuguuccaacuggcggaccuguacgaacccaggggccggaugacccuggccgacaucgagcgcauugccccgcucgaggagggcacccugcccuucaaccuggcggaggcccagcgccagaaggccagcggggacagcgccaggcccguccugcugcagguggccgaguccgcguacagguucggucuggggagcgucgcgggagccgugggugccaccgccguguauccgaucgaccucgugaagacccguaugcagaaucagagguccaccggcagcuucgugggcgagcucauguacaagaacuccuucgacuguuucaagaagguucuccgguacgagggguucuucggccucuaccgggggcugcuaccccagcugcucggcguggcgcccgagaaggccaucaagcucacggucaacgacuuugugcgggacaaguucaugcacaaggacggcagcgucccccuggccgccgagauucuggcaggcggcugcgccggaggcagccaggucaucuuuaccaacccccuggagaucgugaagaucaggcugcaaguggccggggagauuaccaccggaccccgugugagcgcccugagcguggugagggaccuuggcuucuuuggcauauacaagggagccaaggccugcuuucugagggacaucccguuuuccgccauauacuuucccugcuacgcccacgugaaagcgagcuucgccaacgaggacggccaggucagucccggcucccuacugcuggccggagccaucgccgggaugcccgccgccagccuggugacccccgcggacguuaucaagaccaggcugcagguggcggccagggcgggccagaccaccuacagcggcgugaucgacugcuuccgcaagauccugcgggaggaggggcccaaggcccuguggaaaggcgccggggcaaggguguucaggagcagcccccaguucggggugacccugcuuaccuacgaacugcugcagcggugguucuauaucgacuucgggggagucaagcccaugggcuccgagccugugcccaagagcaggaucaaucugcccgcccccaacccagaccacgugggaggguacaaacuggccguggccaccuucgccggaaucgagaacaaguucggccuguaucugccccuguucaaaccguccgucuccaccagcaaggccaucggcgggggccccugauaauaguccauaaaguaggaaacacuacagcuggagccucgguggccaugcuucuugccccuugggccuccccccagccccuccuccccuuccugcacccguaccccccgcauuauuacucacgguacgaguggucuuugaauaaagucugagugggcggc

SEQ ID NO: 134 - protein, 675 aa, Artificial Sequence; identical to SEQ ID NO: 1
  Construct #2 Amino acid sequence of Citrin gene

SEQ ID NO: 135 - RNA, 2025 nt, Artificial Sequence
  Construct #3 ORF of Citrin gene
auggccgccgccaaggucgcacucaccaaacgggccgaccccgccgagcucaggaccaucuuccucaaguacgccagcaucgagaagaacggggaguucuucaugagccccaacgacuucguaaccagguaccucaauaucuucggcgaaagccagcccaacccgaagaccgucgagcuccucuccggggucgucgaucagaccaaggacgggcucaucuccuuccaggaguucguggccuucgaguccguccucugcgccccggacgcccucuucauggucgccuuccaacucuucgauaaggccgggaaaggcgaggugaccuucgaagaugugaagcagguuuucggccagaccacgauccaccagcauauccccuuuaacugggacagcgaguucgugcagcugcacuucggcaaagagaggaagaggcaccucaccuaugccgaauucacacaauuccugcucgagauucagcuggagcaugccaaacaagccuuuguccagcgggacaacgccaggaccggcagggucaccgcgaucgacuuucgcgauaucauggugaccaucaggccccacgugcucacccccuuuguggaggagugccuggucgccgccgccggcgggacgaccagccaccagguguccuucucauacuucaacggguucaacagccugcugaacaacauggagcugauccgcaagaucuacuccacccuggccggcaccaggaaggacguggaagugaccaaggaggaguucguucucgccgcccagaaauucggacaggugaccccgauggagguggacauccucuuccagcuggccgaucucuacgagccccggggcaggaugacgcucgccgacaucgagcgaaucgccccccuggaggaggguacccuucccuucaaccuggccgaggcccagcgacagaaagccagcggcgacagugccaggcccgugcuccugcagguggccgaauccgccuacagauuuggccugggcagcgucgccggcgcagugggcgccaccgccguguacccgaucgaccuggucaagaccaggaugcagaaccagagaagcaccggcuccuuugugggcgagcuuauguacaagaacagcuucgacugcuucaagaagguccugcguuacgagggcuucuucgggcuguaccggggccugcugccgcagcugcuaggcgucgcgcccgagaaggccauuaagcugaccgugaacgacuucguacgggacaaauucaugcacaaggacggcagugugccccuggccgcagagauccuggccgggggcugugccggcgggucccaggugaucuuuacgaacccccuggagauagugaagauccggcugcagguggccggggagaucaccaccggcccccggguguccgcccugagcgucgugagggaucugggguucuuuggcaucuauaagggugccaaggccugcuuccugcgugacauucccuuuagcgccaucuacuuccccugcuacgcccaugucaaggccagcuucgccaacgaagacggacaggugagccccgggucccugcugcuggccggcgccaucgcagggaugccggccgccucacuggugaccccggcggacgugauaaagacgaggcugcagguggccgcccgcgcaggccagaccacguacucgggugugauagacugcuuccggaagauccugagggaagaaggccccaaggcccuguggaagggggccggcgccaggguguuccgcagcagcccccaguucggggucacccugcucacguacgagcuccugcagaggugguucuacaucgacuuuggcggggucaagcccaugggcagugagccggugcccaagagccggaucaaucugcccgcccccaacccugaccacgucggcggguacaaacuggcgguggccaccuucgccggcaucgagaacaaguuuggccuguaccugccgcuguuuaagccguccgugagcaccuccaaggccaucgggggcggccca

SEQ ID NO: 136 - RNA, 2236 nt, Artificial Sequence
  Construct #3 Full Citrin nucleic acid with UTRs
gggaaauaagagagaaaagaagaguaagaagaaauauaagagccaccauggccgccgccaaggucgcacucaccaaacgggccgaccccgccgagcucaggaccaucuuccucaaguacgccagcaucgagaagaacggggaguucuucaugagccccaacgacuucguaaccagguaccucaauaucuucggcgaaagccagcccaacccgaagaccgucgagcuccucuccggggucgucgaucagaccaaggacgggcucaucuccuuccaggaguucguggccuucgaguccguccucugcgccccggacgcccucuucauggucgccuuccaacucuucgauaaggccgggaaaggcgaggugaccuucgaagaugugaagcagguuuucggccagaccacgauccaccagcauauccccuuuaacugggacagcgaguucgugcagcugcacuucggcaaagagaggaagaggcaccucaccuaugccgaauucacacaauuccugcucgagauucagcuggagcaugccaaacaagccuuuguccagcgggacaacgccaggaccggcagggucaccgcgaucgacuuucgcgauaucauggugaccaucaggccccacgugcucacccccuuuguggaggagugccuggucgccgccgccggcgggacgaccagccaccagguguccuucucauacuucaacggguucaacagccugcugaacaacauggagcugauccgcaagaucuacuccacccuggccggcaccaggaaggacguggaagugaccaaggaggaguucguucucgccgcccagaaauucggacaggugaccccgauggagguggacauccucuuccagcuggccgaucucuacgagccccggggcaggaugacgcucgccgacaucgagcgaaucgccccccuggaggaggguacccuucccuucaaccuggccgaggcccagcgacagaaagccagcggcgacagugccaggcccgugcuccugcagguggccgaauccgccuacagauuuggccugggcagcgucgccggcgcagugggcgccaccgccguguacccgaucgaccuggucaagaccaggaugcagaaccagagaagcaccggcuccuuugugggcgagcuuauguacaagaacagcuucgacugcuucaagaagguccugcguuacgagggcuucuucgggcuguaccggggccugcugccgcagcugcuaggcgucgcgcccgagaaggccauuaagcugaccgugaacgacuucguacgggacaaauucaugcacaaggacggcagugugccccuggccgcagagauccuggccgggggcugugccggcgggucccaggugaucuuuacgaacccccuggagauagugaagauccggcugcagguggccggggagaucaccaccggcccccggguguccgcccugagcgucgugagggaucugggguucuuuggcaucuauaagggugccaaggccugcuuccugcgugacauucccuuuagcgccaucuacuuccccugcuacgcccaugucaaggccagcuucgccaacgaagacggacaggugagccccgggucccugcugcuggccggcgccaucgcagggaugccggccgccucacuggugaccccggcggacgugauaaagacgaggcugcagguggccgcccgcgcaggccagaccacguacucgggugugauagacugcuuccggaagauccugagggaagaaggccccaaggcccuguggaagggggccggcgccaggguguuccgcagcagcccccaguucggggucacccugcucacguacgagcuccugcagaggugguucuacaucgacuuuggcggggucaagcccaugggcagugagccggugcccaagagccggaucaaucugcccgcccccaacccugaccacgucggcggguacaaacuggcgguggccaccuucgccggcaucgagaacaaguuuggccuguaccugccgcuguuuaagccguccgugagcaccuccaaggccaucgggggcggcccaugauaauaguccauaaaguaggaaacacuacagcuggagccucgguggccaugcuucuugccccuugggccuccccccagccccuccuccccuuccugcacccguaccccccgcauuauuacucacgguacgaguggucuuugaauaaagucugagugggcggc

SEQ ID NO: 137 - protein, 675 aa, Artificial Sequence; identical to SEQ ID NO: 1
  Construct #3 Amino acid sequence of Citrin gene

SEQ ID NO: 138 - RNA, 2025 nt, Artificial Sequence
  Construct #4 ORF of Citrin gene
auggccgccgcuaaggucgcccucacgaagcgggccgaucccgccgagcuccggaccaucuuucucaaauacgccagcaucgagaagaacggcgaguucuucaugucccccaacgacuucgucaccagguaccuaaacaucuucggcgagagccagccgaaccccaagaccgucgaauugcuaucgggcgucgucgaccagaccaaggacgggcucaucagcuuccaggaguucgucgccuucgaguccguccucugcgcccccgacgcccucuucaugguagcauuccaguuguucgacaaggccggaaagggggaggugaccuucgaggacgugaagcagguguuuggucagaccaccauccaucagcacaucccguuuaacugggacucggaguucgugcagcuccacuucggcaaggaacgaaagcggcaccucaccuacgccgaguucacccaguuccugcuggagauccagcuggaacacgccaagcaggccuucgugcagcgagacaaugcgaggaccgggcgcgugacugccaucgauuucagggacaucauggugaccauccggccccacgugcugacucccuucguggaggagugccuggucgcagccgccggggguaccaccucccaccaggugagcuucagcuacuucaacggcuucaacagccugcucaacaacauggaacugauccgcaagaucuauuccacacucgccggcaccaggaaggauguggaggugaccaaggaggaguuugugcuggcggcccagaaguuugggcaggucacccccauggagguggacauccucuuccagcuggccgaccuguacgagcccaggggcaggaugacccuggccgacaucgaacgaaucgccccccuggaggagggcacacugcccuucaaccuggccgaggcccagaggcagaaggccuccggcgacagcgcccgacccgugcuucugcaaguggccgagagcgccuaccgcuuuggccugggauccguggccggcgccgucggugccaccgccguguacccaaucgaccuagugaagacacgcaugcagaaccagcgcagcaccggcuccuuugucggggagcugauguauaagaacagcuucgacugcuucaagaaggugcugcgcuacgagggcuucuucggccuguacagggggcugcugccccaacugcugggcguggcccccgagaaggccaucaagcugaccguuaacgacuucgugcgagacaaguucaugcacaaggacggcagcgugcccuuggccgcagagauacuggccgggggcugcgccggcgggucgcaggugaucuucaccaacccccucgagaucguaaagaucaggcuccaaguggccggggagaucaccaccggccccaggguguccgcccugucgguggucagggaccugggguucuucgggauauacaagggcgcgaaggccugcuuccugagggacauccccuucagcgccaucuacuuucccugcuacgcccacgucaaggccagcuucgccaacgaggauggccagguguccccgggcucccugcuccuggccggugcuaucgcgggaaugcccgccgcgagccuggugacccccgccgaugugaucaagaccaggcugcaagucgcggcgagggccggucagaccaccuacuccggggucaucgauugcuuuaggaagauccuccgggaggaggggcccaaggcacuguggaagggggccggggccaggguguuccguagcuccccccaguuuggcgugacccugcugaccuacgaacugcugcagaggugguucuacaucgacuucgggggcgugaagcccaugggcuccgagccggugccuaagagccggaucaaucugcccgcccccaaccccgaccacguggggggcuacaagcuggccguggcuaccuucgccgguaucgagaacaaguucggccuguaccugccccuguucaagcccuccgugagcacgagcaaggccaucgggggcggcccc

SEQ ID NO: 139 - RNA, 2236 nt, Artificial Sequence
  Construct #4 Full Citrin nucleic acid with UTRs
gggaaauaagagagaaaagaagaguaagaagaaauauaagagccaccauggccgccgcuaaggucgcccucacgaagcgggccgaucccgccgagcuccggaccaucuuucucaaauacgccagcaucgagaagaacggcgaguucuucaugucccccaacgacuucgucaccagguaccuaaacaucuucggcgagagccagccgaaccccaagaccgucgaauugcuaucgggcgucgucgaccagaccaaggacgggcucaucagcuuccaggaguucgucgccuucgaguccguccucugcgcccccgacgcccucuucaugguagcauuccaguuguucgacaaggccggaaagggggaggugaccuucgaggacgugaagcagguguuuggucagaccaccauccaucagcacaucccguuuaacugggacucggaguucgugcagcuccacuucggcaaggaacgaaagcggcaccucaccuacgccgaguucacccaguuccugcuggagauccagcuggaacacgccaagcaggccuucgugcagcgagacaaugcgaggaccgggcgcgugacugccaucgauuucagggacaucauggugaccauccggccccacgugcugacucccuucguggaggagugccuggucgcagccgccggggguaccaccucccaccaggugagcuucagcuacuucaacggcuucaacagccugcucaacaacauggaacugauccgcaagaucuauuccacacucgccggcaccaggaaggauguggaggugaccaaggaggaguuugugcuggcggcccagaaguuugggcaggucacccccauggagguggacauccucuuccagcuggccgaccuguacgagcccaggggcaggaugacccuggccgacaucgaacgaaucgccccccuggaggagggcacacugcccuucaaccuggccgaggcccagaggcagaaggccuccggcgacagcgcccgacccgugcuucugcaaguggccgagagcgccuaccgcuuuggccugggauccguggccggcgccgucggugccaccgccguguacccaaucgaccuagugaagacacgcaugcagaaccagcgcagcaccggcuccuuugucggggagcugauguauaagaacagcuucgacugcuucaagaaggugcugcgcuacgagggcuucuucggccuguacagggggcugcugccccaacugcugggcguggcccccgagaaggccaucaagcugaccguuaacgacuucgugcgagacaaguucaugcacaaggacggcagcgugcccuuggccgcagagauacuggccgggggcugcgccggcgggucgcaggugaucuucaccaacccccucgagaucguaaagaucaggcuccaaguggccggggagaucaccaccggccccaggguguccgcccugucgguggucagggaccugggguucuucgggauauacaagggcgcgaaggccugcuuccugagggacauccccuucagcgccaucuacuuucccugcuacgcccacgucaaggccagcuucgccaacgaggauggccagguguccccgggcucccugcuccuggccggugcuaucgcgggaaugcccgccgcgagccuggugacccccgccgaugugaucaagaccaggcugcaagucgcggcgagggccggucagaccaccuacuccggggucaucgauugcuuuaggaagauccuccgggaggaggggcccaaggcacuguggaagggggccggggccaggguguuccguagcuccccccaguuuggcgugacccugcugaccuacgaacugcugcagaggugguucuacaucgacuucgggggcgugaagcccaugggcuccgagccggugccuaagagccggaucaaucugcccgcccccaaccccgaccacguggggggcuacaagcuggccguggcuaccuucgccgguaucgagaacaaguucggccuguaccugccccuguucaagcccuccgugagcacgagcaaggccaucgggggcggccccugauaauaguccauaaaguaggaaacacuacagcuggagccucgguggccaugcuucuugccccuugggccuccccccagccccuccuccccuuccugcacccguaccccccgcauuauuacucacgguacgaguggucuuugaauaaagucugagugggcggc

SEQ ID NO: 140 - protein, 675 aa, Artificial Sequence; identical to SEQ ID NO: 1
  Construct #4 Amino acid sequence of Citrin gene

SEQ ID NO: 141 - RNA, 70 nt, Artificial Sequence; identical to SEQ ID NO: 121
  mRNA encoding non-translated Factor IX (NTFIX

SEQ ID NO: 142 - RNA, 85 nt, Artificial Sequence
  miR-126
cgcuggcgacgggacauuauuacuuuugguacgcgcugugacacuucaaacucguaccgugaguaauaaugcgccguccacggca

SEQ ID NO: 143 - RNA, 22 nt, Artificial Sequence
  miR-126-3p
ucguaccgugaguaauaaugcg

SEQ ID NO: 144 - RNA, 22 nt, Artificial Sequence
  miR-126-3p binding site
cgcauuauuacucacgguacga

SEQ ID NO: 145 - RNA, 21 nt, Artificial Sequence
  miR-126-5p
cauuauuacuuuugguacgcg

SEQ ID NO: 146 - RNA, 21 nt, Artificial Sequence
  miR-126-5p binding site
cgcguaccaaaaguaauaaug

SEQ ID NO: 147 - RNA, 166 nt, Artificial Sequence
  3' UTR with miR 142-3p and miR 126-3p binding sites variant 2
ugauaauaguccauaaaguaggaaacacuacagcuggagccucgguggccuagcuucuugccccuugggccuccccccagccccuccuccccuuccugcacccguaccccccgcauuauuacucacgguacgaguggucuuugaauaaagucugagugggcggcsd

SEQ ID NO: 148 - RNA, 142 nt, Artificial Sequence
  3' UTR with miR 142-3p binding site variant 2
ugauaauaggcuggagccucgguggccuagcuucuugccccuugggccuccccccagccccuccuccccuuccugcacccguacccccuccauaaaguaggaaacacuacaguggucuuugaauaaagucugagugggcggc

SEQ ID NO: 149 - RNA, 119 nt, Artificial Sequence
  3' UTR, no miR binding sites variant 2
ugauaauaggcuggagccucgguggccuagcuucuugccccuugggccuccccccagccccuccuccccuuccugcacccguacccccguggucuuugaauaaagucugagugggcggc

SEQ ID NO: 150 - RNA, 141 nt, Artificial Sequence
  3' UTR with miR 126-3p binding site variant 3
ugauaauaggcuggagccucgguggccuagcuucuugccccuugggccuccccccagccccuccuccccuuccugcacccguaccccccgcauuauuacucacgguacgaguggucuuugaauaaagucugagugggcggc

SEQ ID NO: 151 - RNA, 188 nt, Artificial Sequence
  3' UTR with 3 miR 142-3p binding sites variant 2
ugauaauaguccauaaaguaggaaacacuacagcuggagccucgguggccuagcuucuugccccuugggccuccauaaaguaggaaacacuacauccccccagccccuccuccccuuccugcacccguacccccuccauaaaguaggaaacacuacaguggucuuugaauaaagucugagugggcggc

SEQ ID NO: 152 - RNA, 142 nt, Artificial Sequence
  3'UTR with miR 142-3p binding site, P1 insertion variant 2
ugauaauaguccauaaaguaggaaacacuacagcuggagccucgguggccuagcuucuugccccuugggccuccccccagccccuccuccccuuccugcacccguacccccguggucuuugaauaaagucugagugggcggc

SEQ ID NO: 153 - RNA, 142 nt, Artificial Sequence
  3'UTR with miR 142-3p binding site, P2 insertion variant 2
ugauaauaggcuggagccucgguggcuccauaaaguaggaaacacuacacuagcuucuugccccuugggccuccccccagccccuccuccccuuccugcacccguacccccguggucuuugaauaaagucugagugggcggc

SEQ ID NO: 154 - RNA, 142 nt, Artificial Sequence
  3'UTR with miR 142-3p binding site, P3 insertion variant 2
ugauaauaggcuggagccucgguggccuagcuucuugccccuugggccuccauaaaguaggaaacacuacauccccccagccccuccuccccuuccugcacccguacccccguggucuuugaauaaagucugagugggcggc

SEQ ID NO: 155 - RNA, 142 nt, Artificial Sequence
  3'UTR with miR 155-5p binding site variant 2
ugauaauaggcuggagccucgguggccuagcuucuugccccuugggccuccccccagccccuccuccccuuccugcacccguacccccaccccuaucacaauuagcauuaaguggucuuugaauaaagucugagugggcggc

SEQ ID NO: 156 - RNA, 188 nt, Artificial Sequence
  3' UTR with 3 miR 155-5p binding sites variant 2
ugauaauagaccccuaucacaauuagcauuaagcuggagccucgguggccuagcuucuugccccuugggccaccccuaucacaauuagcauuaauccccccagccccuccuccccuuccugcacccguacccccaccccuaucacaauuagcauuaaguggucuuugaauaaagucugagugggcggc

SEQ ID NO: 157 - RNA, 188 nt, Artificial Sequence
  3'UTR with 2 miR 155-5p binding sites and 1 miR 142-3p binding site variant 2
ugauaauagaccccuaucacaauuagcauuaagcuggagccucgguggccuagcuucuugccccuugggccuccauaaaguaggaaacacuacauccccccagccccuccuccccuuccugcacccguacccccaccccuaucacaauuagcauuaaguggucuuugaauaaagucugagugggcggc